European Patent Specification EP 3 746 467 B1, published October 8, 2025. Title: MODIFIED LIPIDATED RELAXIN B CHAIN PEPTIDES AND THEIR THERAPEUTIC USE. Applicant: SANOFI. The sequence listing filed with the application follows.

SEQUENCE LISTING (104 sequences)

SEQ ID NO: 1 - protein, 24 aa, Artificial Sequence
  Peptide analogue of the B-chain of Relaxin-2
  Peptide analogue of the B-chain of Relaxin-2
  VARIANT 1: The peptide is substituted with an acetyl (Ac) group on its N-terminal extremity
  VARIANT 10: Xaa in position 10 represents 2-amino-4-acetamido-hexanoic acid (Nε-Acetyl-lysine - K(Ac))
  VARIANT 12: Xaa in position 12 represents 2-amino-isobutyric acid (Aib)
  VARIANT 13: Xaa in position 13 represents 2-amino-isobutyric acid (Aib)
  VARIANT 16: Xaa in position 16 represents a lysine amino acid bound on the nitrogen atom of its lateral chain to a -(TTDS)3-(gamma glutamic acid)3-Palmitoyl group (-(TTDS)3-(gE)3-Palm)
  VARIANT 21: Xaa in position 21 represents 2-amino-isobutyric acid (Aib)
  VARIANT 24: Xaa in position 24 represents 2-amino-4-acetamido-hexanoic acid (Nε-Acetyl-lysine - K(Ac))
  VARIANT 24: The peptide is substituted with an –NH2 group on its C-terminal extremity
LEGREKVRAXIXXEGXSTWSXRKX

SEQ ID NO: 2 - protein, 24 aa, Artificial Sequence
  Peptide analogue of the B-chain of Relaxin-2
  Peptide analogue of the B-chain of Relaxin-2
  VARIANT 1: The peptide is substituted with an acetyl (Ac) group on its N-terminal extremity
  VARIANT 10: Xaa in position 10 represents 2-amino-4-acetamido-hexanoic acid (Nε-Acetyl-lysine - K(Ac))
  VARIANT 12: Xaa in position 12 represents 2-amino-isobutyric acid (Aib)
  VARIANT 13: Xaa in position 13 represents 2-amino-isobutyric acid (Aib)
  VARIANT 16: Xaa in position 16 represents a lysine amino acid bound on the nitrogen atom of its lateral chain to a -(TTDS)3-(gamma glutamic acid)3-Palmitoyl group (-(TTDS)3-(gE)3-Palm)
  VARIANT 21: Xaa in position 21 represents 2-amino-isobutyric acid (Aib)
  VARIANT 24: Xaa in position 24 represents 2-amino-4-acetamido-hexanoic acid (Nε-Acetyl-lysine - K(Ac))
  VARIANT 24: The peptide is substituted with an –NH2 group on its C-terminal extremity
LEGREKVRAXIXXEGXSTFSXRAX

SEQ ID NO: 3 - protein, 24 aa, Artificial Sequence
  Peptide analogue of the B-chain of Relaxin-2
  Peptide analogue of the B-chain of Relaxin-2
  VARIANT 1: The peptide is substituted with an acetyl (Ac) group on its N-terminal extremity
  VARIANT 10: Xaa in position 10 represents 2-amino-4-acetamido-hexanoic acid (Nε-Acetyl-lysine - K(Ac))
  VARIANT 12: Xaa in position 12 represents 2-amino-isobutyric acid (Aib)
  VARIANT 13: Xaa in position 13 represents 2-amino-isobutyric acid (Aib)
  VARIANT 16: Xaa in position 16 represents a lysine amino acid bound on the nitrogen atom of its lateral chain to a -(TTDS)3-(gamma glutamic acid)3-Palmitoyl group (-(TTDS)3-(gE)3-Palm)
  VARIANT 21: Xaa in position 21 represents α-Methyl-lysine (Mly)
  VARIANT 24: The peptide is substituted with an –NH2 group on its C-terminal extremity
  VARIANT 24: Xaa in position 24 represents 2-amino-4-acetamido-hexanoic acid (Nε-Acetyl-lysine - K(Ac))
LEGREKVRAXIXXEGXSTFSXRAX

SEQ ID NO: 4 - protein, 24 aa, Artificial Sequence
  Peptide analogue of the B-chain of Relaxin-2
  Peptide analogue of the B-chain of Relaxin-2
  VARIANT 1: The peptide is substituted with an acetyl (Ac) group on its N-terminal extremity
  VARIANT 10: Xaa in position 10 represents 2-amino-4-acetamido-hexanoic acid (Nε-Acetyl-lysine - K(Ac))
  VARIANT 12: Xaa in position 12 represents 2-amino-isobutyric acid (Aib)
  VARIANT 13: Xaa in position 13 represents 2-amino-isobutyric acid (Aib)
  VARIANT 16: Xaa in position 16 represents a lysine amino acid bound on the nitrogen atom of its lateral chain to a -(TTDS)2-(gamma glutamic acid)3-Palmitoyl group (-(TTDS)2-(gE)3-Palm)
  VARIANT 21: Xaa in position 21 represents 2-amino-isobutyric acid (Aib)
  VARIANT 24: Xaa in position 24 represents 2-amino-4-acetamido-hexanoic acid (Nε-Acetyl-lysine - K(Ac))
  VARIANT 24: The peptide is substituted with an –NH2 group on its C-terminal extremity
LEGREKVRAXIXXEGXSTWSXRKX

SEQ ID NO: 5 - protein, 24 aa, Artificial Sequence
  Peptide analogue of the B-chain of Relaxin-2
  Peptide analogue of the B-chain of Relaxin-2
  VARIANT 1: The peptide is substituted with an acetyl (Ac) group on its N-terminal extremity
  VARIANT 10: Xaa in position 10 represents 2-amino-4-acetamido-hexanoic acid (Nε-Acetyl-lysine - K(Ac))
  VARIANT 12: Xaa in position 12 represents 2-amino-isobutyric acid (Aib)
  VARIANT 13: Xaa in position 13 represents 2-amino-isobutyric acid (Aib)
  VARIANT 16: Xaa in position 16 represents a lysine amino acid bound on the nitrogen atom of its lateral chain to a -(PEG2)4-(gamma glutamic acid)3-Palmitoyl group (-(PEG2)4-(gE)3-Palm)
  VARIANT 21: Xaa in position 21 represents 2-amino-isobutyric acid (Aib)
  VARIANT 24: The peptide is substituted with an –NH2 group on its C-terminal extremity
  VARIANT 24: Xaa in position 24 represents 2-amino-4-acetamido-hexanoic acid (Nε-Acetyl-lysine - K(Ac))
LEGREKVRAXIXXEGXSTWSXRKX

SEQ ID NO: 6 - protein, 24 aa, Artificial Sequence
  Peptide analogue of the B-chain of Relaxin-2
  Peptide analogue of the B-chain of Relaxin-2
  VARIANT 1: The peptide is substituted with an acetyl (Ac) group on its N-terminal extremity
  VARIANT 10: Xaa in position 10 represents 2-amino-4-acetamido-hexanoic acid (Nε-Acetyl-lysine - K(Ac))
  VARIANT 12: Xaa in position 12 represents 2-amino-isobutyric acid (Aib)
  VARIANT 13: Xaa in position 13 represents 2-amino-isobutyric acid (Aib)
  VARIANT 16: Xaa in position 16 represents a lysine amino acid bound on the nitrogen atom of its lateral chain to a -(TTDS)2-(gamma glutamic acid)3-Stearoyl group (-(TTDS)2-(gE)3-Stea)
  VARIANT 21: Xaa in position 21 represents 2-amino-isobutyric acid (Aib)
  VARIANT 24: Xaa in position 24 represents 2-amino-4-acetamido-hexanoic acid (Nε-Acetyl-lysine - K(Ac))
  VARIANT 24: The peptide is substituted with an –NH2 group on its C-terminal extremity
LEGREKVRAXIXXEGXSTWSXRKX

SEQ ID NO: 7 - protein, 24 aa, Artificial Sequence
  Peptide analogue of the B-chain of Relaxin-2
  Peptide analogue of the B-chain of Relaxin-2
  VARIANT 1: The peptide is substituted with an acetyl (Ac) group on its N-terminal extremity
  VARIANT 10: Xaa in position 10 represents 2-amino-4-acetamido-hexanoic acid (Nε-Acetyl-lysine - K(Ac))
  VARIANT 12: Xaa in position 12 represents 2-amino-isobutyric acid (Aib)
  VARIANT 13: Xaa in position 13 represents 2-amino-isobutyric acid (Aib)
  VARIANT 16: Xaa in position 16 represents a lysine amino acid bound on the nitrogen atom of its lateral chain to a -(TTDS)3-(gamma glutamic acid)3-Stearoyl group (-(TTDS)3-(gE)3-Stea)
  VARIANT 21: Xaa in position 21 represents α-Methyl-lysine (Mly)
  VARIANT 24: Xaa in position 24 represents 2-amino-4-acetamido-hexanoic acid (Nε-Acetyl-lysine - K(Ac))
  VARIANT 24: The peptide is substituted with an –NH2 group on its C-terminal extremity
LEGREKVRAXIXXEGXSTFSXRAX

SEQ ID NO: 8 - protein, 24 aa, Artificial Sequence
  Peptide analogue of the B-chain of Relaxin-2
  Peptide analogue of the B-chain of Relaxin-2
  VARIANT 1: The peptide is substituted with an acetyl (Ac) group on its N-terminal extremity
  VARIANT 10: Xaa in position 10 represents 2-amino-4-acetamido-hexanoic acid (Nε-Acetyl-lysine - K(Ac))
  VARIANT 12: Xaa in position 12 represents 2-amino-isobutyric acid (Aib)
  VARIANT 13: Xaa in position 13 represents 2-amino-isobutyric acid (Aib)
  VARIANT 16: Xaa in position 16 represents a lysine amino acid bound on the nitrogen atom of its lateral chain to a -(PEG2)4-(gamma glutamic acid)3-Palmitoyl group (-(PEG2)4-(gE)3-Palm)
  VARIANT 21: Xaa in position 21 represents α-Methyl-lysine (Mly)
  VARIANT 24: Xaa in position 24 represents 2-amino-4-acetamido-hexanoic acid (Nε-Acetyl-lysine - K(Ac))
  VARIANT 24: The peptide is substituted with an –NH2 group on its C-terminal extremity
LEGREKVRAXIXXEGXSTFSXRAX

SEQ ID NO: 9 - protein, 24 aa, Artificial Sequence
  Peptide analogue of the B-chain of Relaxin-2
  Peptide analogue of the B-chain of Relaxin-2
  VARIANT 1: The peptide is substituted with an acetyl (Ac) group on its N-terminal extremity
  VARIANT 10: Xaa in position 10 represents 2-amino-4-acetamido-hexanoic acid (Nε-Acetyl-lysine - K(Ac))
  VARIANT 12: Xaa in position 12 represents 2-amino-isobutyric acid (Aib)
  VARIANT 13: Xaa in position 13 represents 2-amino-isobutyric acid (Aib)
  VARIANT 16: Xaa in position 16 represents a lysine amino acid bound on the nitrogen atom of its lateral chain to a -(TTDS)2-(gamma glutamic acid)2-Palmitoyl group (-(TTDS)2-(gE)2-Palm)
  VARIANT 21: Xaa in position 21 represents α-Methyl-lysine (Mly)
  VARIANT 24: Xaa in position 24 represents 2-amino-4-acetamido-hexanoic acid (Nε-Acetyl-lysine - K(Ac))
  VARIANT 24: The peptide is substituted with an –NH2 group on its C-terminal extremity
LEGREKVRAXIXXEGXSTFSXRAX

SEQ ID NO: 10 - protein, 24 aa, Artificial Sequence
  Peptide analogue of the B-chain of Relaxin-2
  Peptide analogue of the B-chain of Relaxin-2
  VARIANT 1: The peptide is substituted with an acetyl (Ac) group on its N-terminal extremity
  VARIANT 10: Xaa in position 10 represents 2-amino-4-acetamido-hexanoic acid (Nε-Acetyl-lysine - K(Ac))
  VARIANT 12: Xaa in position 12 represents 2-amino-isobutyric acid (Aib)
  VARIANT 13: Xaa in position 13 represents 2-amino-isobutyric acid (Aib)
  VARIANT 16: Xaa in position 16 represents a lysine amino acid bound on the nitrogen atom of its lateral chain to a -(TTDS)2-(gamma glutamic acid)4-Palmitoyl group (-(TTDS)2-(gE)4-Palm)
  VARIANT 21: Xaa in position 21 represents α-Methyl-lysine (Mly)
  VARIANT 24: Xaa in position 24 represents 2-amino-4-acetamido-hexanoic acid (Nε-Acetyl-lysine - K(Ac))
  VARIANT 24: The peptide is substituted with an –NH2 group on its C-terminal extremity
LEGREKVRAXIXXEGXSTFSXRAX

SEQ ID NO: 11 - protein, 24 aa, Artificial Sequence
  Peptide analogue of the B-chain of Relaxin-2
  Peptide analogue of the B-chain of Relaxin-2
  VARIANT 1: The peptide is substituted with an acetyl (Ac) group on its N-terminal extremity
  VARIANT 10: Xaa in position 10 represents 2-amino-4-acetamido-hexanoic acid (Nε-Acetyl-lysine - K(Ac))
  VARIANT 12: Xaa in position 12 represents 2-amino-isobutyric acid (Aib)
  VARIANT 13: Xaa in position 13 represents 2-amino-isobutyric acid (Aib)
  VARIANT 16: Xaa in position 16 represents a lysine amino acid bound on the nitrogen atom of its lateral chain to a -(TTDS)3-(gamma glutamic acid)3-Palmitoyl group (-(TTDS)3-(gE)3-Palm)
  VARIANT 21: Xaa in position 21 represents α-Methyl-lysine (Mly)
  VARIANT 24: Xaa in position 24 represents 2-amino-4-acetamido-hexanoic acid (Nε-Acetyl-lysine - K(Ac))
  VARIANT 24: The peptide is substituted with an –NH2 group on its C-terminal extremity
LEGREKVRAXIXXEGXSTWSXRAX

SEQ ID NO: 12 - protein, 24 aa, Artificial Sequence
  Peptide analogue of the B-chain of Relaxin-2
  Peptide analogue of the B-chain of Relaxin-2
  VARIANT 1: The peptide is substituted with an acetyl (Ac) group on its N-terminal extremity
  VARIANT 10: Xaa in position 10 represents Citruline (Cit)
  VARIANT 12: Xaa in position 12 represents 2-amino-isobutyric acid (Aib)
  VARIANT 13: Xaa in position 13 represents 2-amino-isobutyric acid (Aib)
  VARIANT 16: Xaa in position 16 represents a lysine amino acid bound on the nitrogen atom of its lateral chain to a -(TTDS)3-(gamma glutamic acid)3-Palmitoyl group (-(TTDS)3-(gE)3-Palm)
  VARIANT 21: Xaa in position 21 represents α-Methyl-lysine (Mly)
  VARIANT 24: Xaa in position 24 represents 2-amino-4-acetamido-hexanoic acid (Nε-Acetyl-lysine - K(Ac))
  VARIANT 24: The peptide is substituted with an –NH2 group on its C-terminal extremity
LEGREKVRAXIXXEGXSTFSXRAX

SEQ ID NO: 13 - protein, 24 aa, Artificial Sequence
  Peptide analogue of the B-chain of Relaxin-2
  Peptide analogue of the B-chain of Relaxin-2
  VARIANT 1: The peptide is substituted with an acetyl (Ac) group on its N-terminal extremity
  VARIANT 10: Xaa in position 10 represents 2-amino-4-acetamido-hexanoic acid (Nε-Acetyl-lysine - K(Ac))
  VARIANT 12: Xaa in position 12 represents 2-amino-isobutyric acid (Aib)
  VARIANT 13: Xaa in position 13 represents 2-amino-isobutyric acid (Aib)
  VARIANT 16: Xaa in position 16 represents a lysine amino acid bound on the nitrogen atom of its lateral chain to a -(TTDS)3-(gamma glutamic acid)3-Palmitoyl group (-(TTDS)3-(gE)3-Palm)
  VARIANT 24: Xaa in position 24 represents 2-amino-4-acetamido-hexanoic acid (Nε-Acetyl-lysine - K(Ac))
  VARIANT 24: The peptide is substituted with an –NH2 group on its C-terminal extremity
LEGREKVRAXIXXEGXSTFSKRAX

SEQ ID NO: 14 - protein, 24 aa, Artificial Sequence
  Peptide analogue of the B-chain of Relaxin-2
  Peptide analogue of the B-chain of Relaxin-2
  VARIANT 1: The peptide is substituted with an acetyl (Ac) group on its N-terminal extremity
  VARIANT 10: Xaa in position 10 represents 2-amino-4-acetamido-hexanoic acid (Nε-Acetyl-lysine - K(Ac))
  VARIANT 12: Xaa in position 12 represents 2-amino-isobutyric acid (Aib)
  VARIANT 13: Xaa in position 13 represents 2-amino-isobutyric acid (Aib)
  VARIANT 16: Xaa in position 16 represents a lysine amino acid bound on the nitrogen atom of its lateral chain to a -(TTDS)3-(gamma glutamic acid)3-Palmitoyl group (-(TTDS)3-(gE)3-Palm)
  VARIANT 20: Xaa in position 20 represents D-serine (Dser)
  VARIANT 24: Xaa in position 24 represents 2-amino-4-acetamido-hexanoic acid (Nε-Acetyl-lysine - K(Ac))
  VARIANT 24: The peptide is substituted with an –NH2 group on its C-terminal extremity
LEGREKVRAXIXXEGXSTFXKRAX

SEQ ID NO: 15 - protein, 24 aa, Artificial Sequence
  Peptide analogue of the B-chain of Relaxin-2
  Peptide analogue of the B-chain of Relaxin-2
  VARIANT 1: The peptide is substituted with an acetyl (Ac) group on its N-terminal extremity
  VARIANT 10: Xaa in position 10 represents 2-amino-4-acetamido-hexanoic acid (Nε-Acetyl-lysine - K(Ac))
  VARIANT 12: Xaa in position 12 represents 2-amino-isobutyric acid (Aib)
  VARIANT 13: Xaa in position 13 represents 2-amino-isobutyric acid (Aib)
  VARIANT 16: Xaa in position 16 represents a lysine amino acid bound on the nitrogen atom of its lateral chain to a -(TTDS)3-(gamma glutamic acid)3-Palmitoyl group (-(TTDS)3-(gE)3-Palm)
  VARIANT 20: Xaa in position 20 represents 2-amino-isobutyric acid (Aib)
  VARIANT 24: Xaa in position 24 represents 2-amino-4-acetamido-hexanoic acid (Nε-Acetyl-lysine - K(Ac))
  VARIANT 24: The peptide is substituted with an –NH2 group on its C-terminal extremity
LEGREKVRAXIXXEGXSTFXKRAX

SEQ ID NO: 16 - protein, 24 aa, Artificial Sequence
  Peptide analogue of the B-chain of Relaxin-2
  Peptide analogue of the B-chain of Relaxin-2
  VARIANT 1: The peptide is substituted with an acetyl (Ac) group on its N-terminal extremity
  VARIANT 10: Xaa in position 10 represents 2-amino-4-acetamido-hexanoic acid (Nε-Acetyl-lysine - K(Ac))
  VARIANT 12: Xaa in position 12 represents 2-amino-isobutyric acid (Aib)
  VARIANT 13: Xaa in position 13 represents 2-amino-isobutyric acid (Aib)
  VARIANT 16: Xaa in position 16 represents a lysine amino acid bound on the nitrogen atom of its lateral chain to a -(TTDS)2-(gamma glutamic acid)3-Palmitoyl group (-(TTDS)2-(gE)3-Palm)
  VARIANT 21: Xaa in position 21 represents D-lysine (Dlys)
  VARIANT 24: Xaa in position 24 represents 2-amino-4-acetamido-hexanoic acid (Nε-Acetyl-lysine - K(Ac))
  VARIANT 24: The peptide is substituted with an –NH2 group on its C-terminal extremity
LEGREKVRAXIXXEGXSTFSXRAX

SEQ ID NO: 17 - protein, 24 aa, Artificial Sequence
  Peptide analogue of the B-chain of Relaxin-2
  Peptide analogue of the B-chain of Relaxin-2
  VARIANT 1: The peptide is substituted with an acetyl (Ac) group on its N-terminal extremity
  VARIANT 10: Xaa in position 10 represents 2-amino-4-acetamido-hexanoic acid (Nε-Acetyl-lysine - K(Ac))
  VARIANT 12: Xaa in position 12 represents 2-amino-isobutyric acid (Aib)
  VARIANT 13: Xaa in position 13 represents 2-amino-isobutyric acid (Aib)
  VARIANT 16: Xaa in position 16 represents a lysine amino acid bound on the nitrogen atom of its lateral chain to a -(TTDS)2-(gamma glutamic acid)3-Palmitoyl group (-(TTDS)2-(gE)3-Palm)
  VARIANT 21: Xaa in position 21 represents D-lysine (Dlys)
  VARIANT 24: Xaa in position 24 represents 2-amino-4-acetamido-hexanoic acid (Nε-Acetyl-lysine - K(Ac))
  VARIANT 24: The peptide is substituted with an –NH2 group on its C-terminal extremity
LEGREKVRAXIXXEGXSTWSXRAX

SEQ ID NO: 18 - protein, 24 aa, Artificial Sequence
  Peptide analogue of the B-chain of Relaxin-2
  Peptide analogue of the B-chain of Relaxin-2
  VARIANT 1: The peptide is substituted with an acetyl (Ac) group on its N-terminal extremity
  VARIANT 10: Xaa in position 10 represents 2-amino-4-acetamido-hexanoic acid (Nε-Acetyl-lysine - K(Ac))
  VARIANT 12: Xaa in position 12 represents 2-amino-isobutyric acid (Aib)
  VARIANT 13: Xaa in position 13 represents 2-amino-isobutyric acid (Aib)
  VARIANT 16: Xaa in position 16 represents a lysine amino acid bound on the nitrogen atom of its lateral chain to a -(TTDS)2-(gamma glutamic acid)3-Palmitoyl group (-(TTDS)2-(gE)3-Palm)
  VARIANT 21: Xaa in position 21 represents D-lysine (Dlys)
  VARIANT 24: Xaa in position 24 represents 2-amino-4-acetamido-hexanoic acid (Nε-Acetyl-lysine - K(Ac))
  VARIANT 24: The peptide is substituted with an –NH2 group on its C-terminal extremity
LEGREKVRAXIXXEGXSTWSXRKX

SEQ ID NO: 19 - protein, 24 aa, Artificial Sequence
  Peptide analogue of the B-chain of Relaxin-2
  Peptide analogue of the B-chain of Relaxin-2
  VARIANT 1: The peptide is substituted with an acetyl (Ac) group on its N-terminal extremity
  VARIANT 10: Xaa in position 10 represents 2-amino-4-acetamido-hexanoic acid (Nε-Acetyl-lysine - K(Ac))
  VARIANT 12: Xaa in position 12 represents 2-amino-isobutyric acid (Aib)
  VARIANT 13: Xaa in position 13 represents 2-amino-isobutyric acid (Aib)
  VARIANT 16: Xaa in position 16 reprsents a lysine amino acid bound on the nitrogen atom of its lateral chain to a -(PEG2)3-(gamma glutamic acid)3-Palmitoyl group (-(PEG2)3-(gE)3-Palm)
  VARIANT 21: Xaa in position 21 represents 2-amino-isobutyric acid (Aib)
  VARIANT 24: Xaa in position 24 represents 2-amino-4-acetamido-hexanoic acid (Nε-Acetyl-lysine - K(Ac))
  VARIANT 24: The peptide is substituted with an –NH2 group on its C-terminal extremity
LEGREKVRAXIXXEGXSTWSXRKX

SEQ ID NO: 20 - protein, 24 aa, Artificial Sequence
  Peptide analogue of the B-chain of Relaxin-2
  Peptide analogue of the B-chain of Relaxin-2
  VARIANT 1: The peptide is substituted with an acetyl (Ac) group on its N-terminal extremity
  VARIANT 10: Xaa in position 10 represents 2-amino-4-acetamido-hexanoic acid (Nε-Acetyl-lysine - K(Ac))
  VARIANT 12: Xaa in position 12 represents 2-amino-isobutyric acid (Aib)
  VARIANT 13: Xaa in position 13 represents 2-amino-isobutyric acid (Aib)
  VARIANT 16: Xaa in position 16 represents a lysine amino acid bound on the nitrogen atom of its lateral chain to a -(TTDS)3-(gamma glutamic acid)3-Stearoyl group (-(TTDS)3-(gE)3-Stea)
  VARIANT 21: Xaa in position 21 represents 2-amino-isobutyric acid (Aib)
  VARIANT 24: Xaa in position 24 represents 2-amino-4-acetamido-hexanoic acid (Nε-Acetyl-lysine - K(Ac))
  VARIANT 24: The peptide is substituted with an –NH2 group on its C-terminal extremity
LEGREKVRAXIXXEGXSTWSXRKX

SEQ ID NO: 21 - protein, 24 aa, Artificial Sequence
  Peptide analogue of the B-chain of Relaxin-2
  Peptide analogue of the B-chain of Relaxin-2
  VARIANT 1: The peptide is substituted with an acetyl (Ac) group on its N-terminal extremity
  VARIANT 10: Xaa in position 10 represents 2-amino-4-acetamido-hexanoic acid (Nε-Acetyl-lysine - K(Ac))
  VARIANT 12: Xaa in position 12 represents 2-amino-isobutyric acid (Aib)
  VARIANT 13: Xaa in position 13 represents 2-amino-isobutyric acid (Aib)
  VARIANT 16: Xaa in position 16 represents a lysine amino acid bound on the nitrogen atom of its lateral chain to a -(PEG2)4-(gamma glutamic acid)3-Stearoyl group (-(PEG2)4-(gE)3-Stea)
  VARIANT 21: Xaa in position 21 represents 2-amino-isobutyric acid (Aib)
  VARIANT 24: Xaa in position 24 represents 2-amino-4-acetamido-hexanoic acid (Nε-Acetyl-lysine - K(Ac))
  VARIANT 24: The peptide is substituted with an –NH2 group on its C-terminal extremity
LEGREKVRAXIXXEGXSTWSXRKX

SEQ ID NO: 22 - protein, 24 aa, Artificial Sequence
  Peptide analogue of the B-chain of Relaxin-2
  Peptide analogue of the B-chain of Relaxin-2
  VARIANT 1: The peptide is substituted with an acetyl (Ac) group on its N-terminal extremity
  VARIANT 10: Xaa in position 10 represents 2-amino-4-acetamido-hexanoic acid (Nε-Acetyl-lysine - K(Ac))
  VARIANT 12: Xaa in position 12 represents 2-amino-isobutyric acid (Aib)
  VARIANT 13: Xaa in position 13 represents 2-amino-isobutyric acid (Aib)
  VARIANT 16: Xaa in position 16 represents a lysine amino acid bound on the nitrogen atom of its lateral chain to a -(PEG2DGA)3-(gamma glutamic acid)3-Palmitoyl group (-(PEG2DGA)3-(gE)3-Palm)
  VARIANT 21: Xaa in position 21 represents α-Methyl-lysine (Mly)
  VARIANT 24: Xaa in position 24 represents 2-amino-4-acetamido-hexanoic acid (Nε-Acetyl-lysine - K(Ac))
  VARIANT 24: The peptide is substituted with an –NH2 group on its C-terminal extremity
LEGREKVRAXIXXEGXSTFSXRAX

SEQ ID NO: 23 - protein, 24 aa, Artificial Sequence
  Peptide analogue of the B-chain of Relaxin-2
  Peptide analogue of the B-chain of Relaxin-2
  VARIANT 1: The peptide is substituted with an acetyl (Ac) group on its N-terminal extremity
  VARIANT 10: Xaa in position 10 represents 2-amino-4-acetamido-hexanoic acid (Nε-Acetyl-lysine - K(Ac))
  VARIANT 12: Xaa in position 12 represents 2-amino-isobutyric acid (Aib)
  VARIANT 13: Xaa in position 13 represents 2-amino-isobutyric acid (Aib)
  VARIANT 16: Xaa in position 16 represents a lysine amino acid bound on the nitrogen atom of its lateral chain to a -(TTDS)3-(gamma glutamic acid)3-Palmitoyl group (-(TTDS)3-(gE)3-Palm)
  VARIANT 21: Xaa in position 21 represents α-Methyl-lysine (Mly)
  VARIANT 24: Xaa in position 24 represents 2-amino-4-acetamido-hexanoic acid (Nε-Acetyl-lysine - K(Ac))
  VARIANT 24: The peptide is substituted with an –NH2 group on its C-terminal extremity
LEGRELVRAXIXXEGXSTFSXRAX

SEQ ID NO: 24 - protein, 24 aa, Artificial Sequence
  Peptide analogue of the B-chain of Relaxin-2
  Peptide analogue of the B-chain of Relaxin-2
  VARIANT 1: The peptide is substituted with an acetyl (Ac) group on its N-terminal extremity
  VARIANT 10: Xaa in position 10 represents 2-amino-4-acetamido-hexanoic acid (Nε-Acetyl-lysine - K(Ac))
  VARIANT 12: Xaa in position 12 represents 2-amino-isobutyric acid (Aib)
  VARIANT 13: Xaa in position 13 represents 2-amino-isobutyric acid (Aib)
  VARIANT 16: Xaa in position 16 represents a lysine amino acid bound on the nitrogen atom of its lateral chain to a -(TTDS)3-(gamma glutamic acid)3-Palmitoyl group (-(TTDS)3-(gE)3-Palm)
  VARIANT 21: Xaa in position 21 represents α-Methyl-lysine (Mly)
  VARIANT 24: Xaa in position 24 represents 2-amino-4-acetamido-hexanoic acid (Nε-Acetyl-lysine - K(Ac))
  VARIANT 24: The peptide is substituted with an –NH2 group on its C-terminal extremity
LEGREFVRAXIXXEGXSTFSXRAX

SEQ ID NO: 25 - protein, 24 aa, Artificial Sequence
  Peptide analogue of the B-chain of Relaxin-2
  Peptide analogue of the B-chain of Relaxin-2
  VARIANT 1: The peptide is substituted with an acetyl (Ac) group on its N-terminal extremity
  VARIANT 10: Xaa in position 10 represents 2-amino-4-acetamido-hexanoic acid (Nε-Acetyl-lysine - K(Ac))
  VARIANT 12: Xaa in position 12 represents 2-amino-isobutyric acid (Aib)
  VARIANT 13: Xaa in position 13 represents 2-amino-isobutyric acid (Aib)
  VARIANT 16: Xaa in position 16 represents a lysine amino acid bound on the nitrogen atom of its lateral chain to a -(TTDS)3-(gamma glutamic acid)3-Palmitoyl group (-(TTDS)3-(gE)3-Palm)
  VARIANT 21: Xaa in position 21 represents α-Methyl-lysine (Mly)
  VARIANT 24: Xaa in position 24 represents 2-amino-4-acetamido-hexanoic acid (Nε-Acetyl-lysine - K(Ac))
  VARIANT 24: The peptide is substituted with an –NH2 group on its C-terminal extremity
LEGREQVRAXIXXEGXSTFSXRAX

SEQ ID NO: 26 - protein, 24 aa, Artificial Sequence
  Peptide analogue of the B-chain of Relaxin-2
  Peptide analogue of the B-chain of Relaxin-2
  VARIANT 1: The peptide is substituted with an acetyl (Ac) group on its N-terminal extremity
  VARIANT 10: Xaa in position 10 represents 2-amino-4-acetamido-hexanoic acid (Nε-Acetyl-lysine - K(Ac))
  VARIANT 12: Xaa in position 12 represents 2-amino-isobutyric acid (Aib)
  VARIANT 13: Xaa in position 13 represents 2-amino-isobutyric acid (Aib)
  VARIANT 16: Xaa in position 16 represents a lysine amino acid bound on the nitrogen atom of its lateral chain to a -(PEG2)4-(gamma glutamic acid)3-Stearoyl group (-(PEG2)4-(gE)3-Stea)
  VARIANT 21: Xaa in position 21 represents α-Methyl-lysine (Mly)
  VARIANT 24: Xaa in position 24 represents 2-amino-4-acetamido-hexanoic acid (Nε-Acetyl-lysine - K(Ac))
  VARIANT 24: The peptide is substituted with an –NH2 group on its C-terminal extremity
LEGREKVRAXIXXEGXSTFSXRAX

SEQ ID NO: 27 - protein, 24 aa, Artificial Sequence
  Peptide analogue of the B-chain of Relaxin-2
  Peptide analogue of the B-chain of Relaxin-2
  VARIANT 1: The peptide is substituted with an acetyl (Ac) group on its N-terminal extremity
  VARIANT 10: Xaa in position 10 represents 2-amino-4-acetamido-hexanoic acid (Nε-Acetyl-lysine - K(Ac))
  VARIANT 12: Xaa in position 12 represents 2-amino-isobutyric acid (Aib)
  VARIANT 13: Xaa in position 13 represents 2-amino-isobutyric acid (Aib)
  VARIANT 16: Xaa in position 16 represents a lysine amino acid bound on the nitrogen atom of its lateral chain to a -(TTDS)3-(gamma glutamic acid)3-Palmitoyl group (-(TTDS)3-(gE)3-Palm)
  VARIANT 21: Xaa in position 21 represents α-Methyl-lysine (Mly)
  VARIANT 24: Xaa in position 24 represents 2-amino-4-acetamido-hexanoic acid (Nε-Acetyl-lysine - K(Ac))
  VARIANT 24: The peptide is substituted with an –NH2 group on its C-terminal extremity
LEGRERVRAXIXXEGXSTFSXRAX

SEQ ID NO: 28 - protein, 24 aa, Artificial Sequence
  Peptide analogue of the B-chain of Relaxin-2
  Peptide analogue of the B-chain of Relaxin-2
  VARIANT 1: The peptide is substituted with an acetyl (Ac) group on its N-terminal extremity
  VARIANT 6: Xaa in position 6 represents homolysine (Hly)
  VARIANT 10: Xaa in position 10 represents 2-amino-4-acetamido-hexanoic acid (Nε-Acetyl-lysine - K(Ac))
  VARIANT 12: Xaa in position 12 represents 2-amino-isobutyric acid (Aib)
  VARIANT 13: Xaa in position 13 represents 2-amino-isobutyric acid (Aib)
  VARIANT 16: Xaa in position 16 represents a lysine amino acid bound on the nitrogen atom of its lateral chain to a -(TTDS)3-(gamma glutamic acid)3-Palmitoyl group (-(TTDS)3-(gE)3-Palm)
  VARIANT 21: Xaa in position 21 represents α-Methyl-lysine (Mly)
  VARIANT 24: Xaa in position 24 represents 2-amino-4-acetamido-hexanoic acid (Nε-Acetyl-lysine - K(Ac))
  VARIANT 24: The peptide is substituted with an –NH2 group on its C-terminal extremity
LEGREXVRAXIXXEGXSTFSXRAX

SEQ ID NO: 29 - protein, 24 aa, Artificial Sequence
  Peptide analogue of the B-chain of Relaxin-2
  Peptide analogue of the B-chain of Relaxin-2
  VARIANT 1: The peptide is substituted with an acetyl (Ac) group on its N-terminal extremity
  VARIANT 9: Xaa in position 9 represents 2-amino-isobutyric acid (Aib)
  VARIANT 10: Xaa in position 10 represents 2-amino-4-acetamido-hexanoic acid (Nε-Acetyl-lysine - K(Ac))
  VARIANT 12: Xaa in position 12 represents 2-amino-isobutyric acid (Aib)
  VARIANT 13: Xaa in position 13 represents 2-amino-isobutyric acid (Aib)
  VARIANT 16: Xaa in position 16 represents a lysine amino acid bound on the nitrogen atom of its lateral chain to a -(TTDS)3-(gamma glutamic acid)3-Palmitoyl group (-(TTDS)3-(gE)3-Palm)
  VARIANT 21: Xaa in position 21 represents α-Methyl-lysine (Mly)
  VARIANT 24: Xaa in position 24 represents 2-amino-4-acetamido-hexanoic acid (Nε-Acetyl-lysine - K(Ac))
  VARIANT 24: The peptide is substituted with an –NH2 group on its C-terminal extremity
LEGREKVRXXIXXEGXSTFSXRAX

SEQ ID NO: 30 - protein, 24 aa, Artificial Sequence
  Peptide analogue of the B-chain of Relaxin-2
  Peptide analogue of the B-chain of Relaxin-2
  VARIANT 1: The peptide is substituted with an acetyl (Ac) group on its N-terminal extremity
  VARIANT 10: Xaa in position 10 represents 2-amino-4-acetamido-hexanoic acid (Nε-Acetyl-lysine - K(Ac))
  VARIANT 12: Xaa in position 12 represents 2-amino-isobutyric acid (Aib)
  VARIANT 13: Xaa in position 13 represents 2-amino-isobutyric acid (Aib)
  VARIANT 16: Xaa in position 16 represents a lysine amino acid bound on the nitrogen atom of its lateral chain to a -(TTDS)3-(gamma glutamic acid)3-Stearoyl group (-(TTDS)3-(gE)3-Stea)
  VARIANT 21: Xaa in position 21 represents α-Methyl-lysine (Mly)
  VARIANT 24: Xaa in position 24 represents 2-amino-4-acetamido-hexanoic acid (Nε-Acetyl-lysine - K(Ac))
  VARIANT 24: The peptide is substituted with an –NH2 group on its C-terminal extremity
LEGREKVRAXIXXEGXSTWSXRAX

SEQ ID NO: 31 - protein, 24 aa, Artificial Sequence
  Peptide analogue of the B-chain of Relaxin-2
  Peptide analogue of the B-chain of Relaxin-2
  VARIANT 1: The peptide is substituted with an acetyl (Ac) group on its N-terminal extremity
  VARIANT 10: Xaa in position 10 represents 2-amino-4-acetamido-hexanoic acid (Nε-Acetyl-lysine - K(Ac))
  VARIANT 12: Xaa in position 12 represents 2-amino-isobutyric acid (Aib)
  VARIANT 13: Xaa in position 13 represents 2-amino-isobutyric acid (Aib)
  VARIANT 16: Xaa in position 16 represents a lysine amino acid bound on the nitrogen atom of its lateral chain to a -(TTDS)3-(gamma glutamic acid)3-Palmitoyl group (-(TTDS)3-(gE)3-Palm)
  VARIANT 21: Xaa in position 21 represents 2-amino-isobutyric acid (Aib)
  VARIANT 24: Xaa in position 24 represents 2-amino-4-acetamido-hexanoic acid (Nε-Acetyl-lysine - K(Ac))
  VARIANT 24: The peptide is substituted with an –NH2 group on its C-terminal extremity
LEGRERVRAXIXXEGXSTWSXRRX

SEQ ID NO: 32 - protein, 24 aa, Artificial Sequence
  Peptide analogue of the B-chain of Relaxin-2
  Peptide analogue of the B-chain of Relaxin-2
  VARIANT 1: The peptide is substituted with an acetyl (Ac) group on its N-terminal extremity
  VARIANT 10: Xaa in position 10 represents 2-amino-4-acetamido-hexanoic acid (Nε-Acetyl-lysine - K(Ac))
  VARIANT 12: Xaa in position 12 represents 2-amino-isobutyric acid (Aib)
  VARIANT 13: Xaa in position 13 represents 2-amino-isobutyric acid (Aib)
  VARIANT 16: Xaa in position 16 represents a lysine amino acid bound on the nitrogen atom of its lateral chain to a -(PEG2DGA)3-(gamma glutamic acid)3-Stearoyl group (-(PEG2DGA)3-(gE)3-Stea)
  VARIANT 21: Xaa in position 21 represents α-Methyl-lysine (Mly)
  VARIANT 24: Xaa in position 24 represents 2-amino-4-acetamido-hexanoic acid (Nε-Acetyl-lysine - K(Ac))
  VARIANT 24: The peptide is substituted with an –NH2 group on its C-terminal extremity
LEGREKVRAXIXXEGXSTFSXRAX

SEQ ID NO: 33 - protein, 24 aa, Artificial Sequence
  Peptide analogue of the B-chain of Relaxin-2
  Peptide analogue of the B-chain of Relaxin-2
  VARIANT 1: The peptide is substituted with an acetyl (Ac) group on its N-terminal extremity
  VARIANT 10: Xaa in position 10 represents 2-amino-4-acetamido-hexanoic acid (Nε-Acetyl-lysine - K(Ac))
  VARIANT 12: Xaa in position 12 represents 2-amino-isobutyric acid (Aib)
  VARIANT 13: Xaa in position 13 represents 2-amino-isobutyric acid (Aib)
  VARIANT 16: Xaa in position 16 represents a lysine amino acid bound on the nitrogen atom of its lateral chain to a -(TTDS)2-(gamma glutamic acid)3-Palmitoyl group (-(TTDS)2-(gE)3-Palm)
  VARIANT 21: Xaa in position 21 represents α-Methyl-lysine (Mly)
  VARIANT 24: Xaa in position 24 represents 2-amino-4-acetamido-hexanoic acid (Nε-Acetyl-lysine - K(Ac))
  VARIANT 24: The peptide is substituted with an –NH2 group on its C-terminal extremity
LEGREKVRAXIXXEGXSTFSXRAX

SEQ ID NO: 34 - protein, 24 aa, Artificial Sequence
  Peptide analogue of the B-chain of Relaxin-2
  Peptide analogue of the B-chain of Relaxin-2
  VARIANT 1: The peptide is substituted with an acetyl (Ac) group on its N-terminal extremity
  VARIANT 10: Xaa in position 10 represents 2-amino-4-acetamido-hexanoic acid (Nε-Acetyl-lysine - K(Ac))
  VARIANT 12: Xaa in position 12 represents 2-amino-isobutyric acid (Aib)
  VARIANT 13: Xaa in position 13 represents 2-amino-isobutyric acid (Aib)
  VARIANT 16: Xaa in position 16 represents a lysine amino acid bound on the nitrogen atom of its lateral chain to a -(TTDS)2-(gamma glutamic acid)3-Stearoyl group (-(TTDS)2-(gE)3-Stea)
  VARIANT 21: Xaa in position 21 represents α-Methyl-lysine (Mly)
  VARIANT 24: Xaa in position 24 represents 2-amino-4-acetamido-hexanoic acid (Nε-Acetyl-lysine - K(Ac))
  VARIANT 24: The peptide is substituted with an –NH2 group on its C-terminal extremity
LEGREKVRAXIXXEGXSTFSXRAX

SEQ ID NO: 35 - protein, 24 aa, Artificial Sequence
  Peptide analogue of the B-chain of Relaxin-2
  Peptide analogue of the B-chain of Relaxin-2
  VARIANT 1: The peptide is substituted with an acetyl (Ac) group on its N-terminal extremity
  VARIANT 10: Xaa in position 10 represents 2-amino-4-acetamido-hexanoic acid (Nε-Acetyl-lysine - K(Ac))
  VARIANT 12: Xaa in position 12 represents 2-amino-isobutyric acid (Aib)
  VARIANT 13: Xaa in position 13 represents 2-amino-isobutyric acid (Aib)
  VARIANT 16: Xaa in position 16 represents a lysine amino acid bound on the nitrogen atom of its lateral chain to a -(TTDS)3-(gamma glutamic acid)3-Palmitoyl group (-(TTDS)3-(gE)3-Palm)
  VARIANT 20: Xaa in position 20 represents 2-amino-isobutyric acid (Aib)
  VARIANT 24: Xaa in position 24 represents 2-amino-4-acetamido-hexanoic acid (Nε-Acetyl-lysine - K(Ac))
  VARIANT 24: The peptide is substituted with an –NH2 group on its C-terminal extremity
LEGREKVRAXIXXEGXSTWXKRAX

SEQ ID NO: 36 - protein, 24 aa, Artificial Sequence
  Peptide analogue of the B-chain of Relaxin-2
  Peptide analogue of the B-chain of Relaxin-2
  VARIANT 1: The peptide is substituted with an acetyl (Ac) group on its N-terminal extremity
  VARIANT 10: Xaa in position 10 represents 2-amino-4-acetamido-hexanoic acid (Nε-Acetyl-lysine - K(Ac))
  VARIANT 12: Xaa in position 12 represents 2-amino-isobutyric acid (Aib)
  VARIANT 13: Xaa in position 13 represents 2-amino-isobutyric acid (Aib)
  VARIANT 16: Xaa in position 16 represents a lysine amino acid bound on the nitrogen atom of its lateral chain to a -(TTDS)3-(gamma glutamic acid)3-Palmitoyl group (-(TTDS)3-(gE)3-Palm)
  VARIANT 21: Xaa in position 21 represents D-lysine (Dlys)
  VARIANT 24: Xaa in position 24 represents 2-amino-4-acetamido-hexanoic acid (Nε-Acetyl-lysine - K(Ac))
  VARIANT 24: The peptide is substituted with an –NH2 group on its C-terminal extremity
LEGREKVRAXIXXEGXSTFSXRAX

SEQ ID NO: 37 - protein, 24 aa, Artificial Sequence
  Peptide analogue of the B-chain of Relaxin-2
  Peptide analogue of the B-chain of Relaxin-2
  VARIANT 1: The peptide is substituted with an acetyl (Ac) group on its N-terminal extremity
  VARIANT 10: Xaa in position 10 represents 2-amino-4-acetamido-hexanoic acid (Nε-Acetyl-lysine - K(Ac))
  VARIANT 12: Xaa in position 12 represents 2-amino-isobutyric acid (Aib)
  VARIANT 13: Xaa in position 13 represents 2-amino-isobutyric acid (Aib)
  VARIANT 16: Xaa in position 16 represents a lysine amino acid bound on the nitrogen atom of its lateral chain to a -(TTDS)3-(gamma glutamic acid)3-Palmitoyl group (-(TTDS)3-(gE)3-Palm)
  VARIANT 21: Xaa in position 21 represents 2-amino-isobutyric acid (Aib)
  VARIANT 24: Xaa in position 24 represents 2-amino-4-acetamido-hexanoic acid (Nε-Acetyl-lysine - K(Ac))
  VARIANT 24: The peptide is substituted with an –NH2 group on its C-terminal extremity
LEGRELVRAXIXXEGXSTWSXRRX

SEQ ID NO: 38 - protein, 24 aa, Artificial Sequence
  Peptide analogue of the B-chain of Relaxin-2
  Peptide analogue of the B-chain of Relaxin-2
  VARIANT 1: The peptide is substituted with an acetyl (Ac) group on its N-terminal extremity
  VARIANT 10: Xaa in position 10 represents 2-amino-4-acetamido-hexanoic acid (Nε-Acetyl-lysine - K(Ac))
  VARIANT 12: Xaa in position 12 represents 2-amino-isobutyric acid (Aib)
  VARIANT 13: Xaa in position 13 represents 2-amino-isobutyric acid (Aib)
  VARIANT 16: Xaa in position 16 represents a lysine amino acid bound on the nitrogen atom of its lateral chain to a -(PEG2)3-(gamma glutamic acid)3-Palmitoyl group (-(PEG2)3-(gE)3-Palm)
  VARIANT 21: Xaa in position 21 represents α-Methyl-lysine (Mly)
  VARIANT 24: Xaa in position 24 represents 2-amino-4-acetamido-hexanoic acid (Nε-Acetyl-lysine - K(Ac))
  VARIANT 24: The peptide is substituted with an –NH2 group on its C-terminal extremity
LEGREKVRAXIXXEGXSTFSXRAX

SEQ ID NO: 39 - protein, 24 aa, Artificial Sequence
  Peptide analogue of the B-chain of Relaxin-2
  Peptide analogue of the B-chain of Relaxin-2
  VARIANT 1: The peptide is substituted with an acetyl (Ac) group on its N-terminal extremity
  VARIANT 10: Xaa in position 10 represents 2-amino-4-acetamido-hexanoic acid (Nε-Acetyl-lysine - K(Ac))
  VARIANT 12: Xaa in position 12 represents 2-amino-isobutyric acid (Aib)
  VARIANT 13: Xaa in position 13 represents 2-amino-isobutyric acid (Aib)
  VARIANT 16: Xaa in position 16 represents a lysine amino acid bound on the nitrogen atom of its lateral chain to a -(TTDS)3-(gamma glutamic acid)3-Palmitoyl group (-(TTDS)3-(gE)3-Palm)
  VARIANT 21: Xaa in position 21 represents 2-amino-isobutyric acid (Aib)
  VARIANT 24: Xaa in position 24 represents 2-amino-4-acetamido-hexanoic acid (Nε-Acetyl-lysine - K(Ac))
  VARIANT 24: The peptide is substituted with an –NH2 group on its C-terminal extremity
LEGREFVRAXIXXEGXSTWSXRRX

SEQ ID NO: 40 - protein, 24 aa, Artificial Sequence
  Peptide analogue of the B-chain of Relaxin-2
  Peptide analogue of the B-chain of Relaxin-2
  VARIANT 1: The peptide is substituted with an acetyl (Ac) group on its N-terminal extremity
  VARIANT 10: Xaa in position 10 represents 2-amino-4-acetamido-hexanoic acid (Nε-Acetyl-lysine - K(Ac))
  VARIANT 12: Xaa in position 12 represents 2-amino-isobutyric acid (Aib)
  VARIANT 13: Xaa in position 13 represents 2-amino-isobutyric acid (Aib)
  VARIANT 16: Xaa in position 16 represents a lysine amino acid bound on the nitrogen atom of its lateral chain to a -(TTDS)3-(gamma glutamic acid)3-Palmitoyl (-(TTDS)3-(gE)3-Palm)
  VARIANT 21: Xaa in position 21 represents 2-amino-isobutyric acid (Aib)
  VARIANT 24: Xaa in position 24 represents 2-amino-4-acetamido-hexanoic acid (Nε-Acetyl-lysine - K(Ac))
  VARIANT 24: The peptide is substituted with an –NH2 group on its C-terminal extremity
LEGREQVRAXIXXEGXSTWSXRRX

SEQ ID NO: 41 - protein, 24 aa, Artificial Sequence
  Peptide analogue of the B-chain of Relaxin-2
  Peptide analogue of the B-chain of Relaxin-2
  VARIANT 1: The peptide is substituted with an acetyl (Ac) group on its N-terminal extremity
  VARIANT 10: Xaa in position 10 represents 2-amino-4-acetamido-hexanoic acid (Nε-Acetyl-lysine - K(Ac))
  VARIANT 12: Xaa in position 12 represents 2-amino-isobutyric acid (Aib)
  VARIANT 13: Xaa in position 13 represents 2-amino-isobutyric acid (Aib)
  VARIANT 16: Xaa in position 16 represents a lysine amino acid bound on the nitrogen atom of its lateral chain to a -(PEG2DGA)3-(gamma glutamic acid)3-Palmitoyl group (-(PEG2DGA)3-(gE)3-Palm)
  VARIANT 21: Xaa in position 21 represents α-Methyl-lysine (Mly)
  VARIANT 24: Xaa in position 24 represents 2-amino-4-acetamido-hexanoic acid (Nε-Acetyl-lysine - K(Ac))
  VARIANT 24: The peptide is substituted with an –NH2 group on its C-terminal extremity
LEGREKVRAXIXXEGXSTWSXRAX

SEQ ID NO: 42 - protein, 24 aa, Artificial Sequence
  Peptide analogue of the B-chain of Relaxin-2
  Peptide analogue of the B-chain of Relaxin-2
  VARIANT 1: The peptide is substituted with an acetyl (Ac) group on its N-terminal extremity
  VARIANT 10: Xaa in position 10 represents 2-amino-4-acetamido-hexanoic acid (Nε-Acetyl-lysine - K(Ac))
  VARIANT 12: Xaa in position 12 represents 2-amino-isobutyric acid (Aib)
  VARIANT 13: Xaa in position 13 represents 2-amino-isobutyric acid (Aib)
  VARIANT 16: Xaa in position 16 represents a lysine amino acid bound on the nitrogen atom of its lateral chain to a -(PEG2)4-(gamma glutamic acid)3-Palmitoyl group (-(PEG2)4-(gE)3-Palm)
  VARIANT 21: Xaa in position 21 represents α-Methyl-lysine (Mly)
  VARIANT 24: Xaa in position 24 represents 2-amino-4-acetamido-hexanoic acid (Nε-Acetyl-lysine - K(Ac))
  VARIANT 24: The peptide is substituted with an –NH2 group on its C-terminal extremity
LEGREKVRAXIXXEGXSTWSXRAX

SEQ ID NO: 43 - protein, 24 aa, Artificial Sequence
  Peptide analogue of the B-chain of Relaxin-2
  Peptide analogue of the B-chain of Relaxin-2
  VARIANT 1: The peptide is substituted with an acetyl (Ac) group on its N-terminal extremity
  VARIANT 6: Xaa in position 6 represents homolysine (Hly)
  VARIANT 10: Xaa in position 10 represents 2-amino-4-acetamido-hexanoic acid (Nε-Acetyl-lysine - K(Ac))
  VARIANT 12: Xaa in position 12 represents 2-amino-isobutyric acid (Aib)
  VARIANT 13: Xaa in position 13 represents 2-amino-isobutyric acid (Aib)
  VARIANT 16: Xaa in position 16 represents a lysine amino acid bound on the nitrogen atom of its lateral chain to a -(TTDS)3-(gamma glutamic acid)3-Stearoyl group (-(TTDS)3-(gE)3-Stea)
  VARIANT 21: Xaa in position 21 represents α-Methyl-lysine (Mly)
  VARIANT 24: Xaa in position 24 represents 2-amino-4-acetamido-hexanoic acid (Nε-Acetyl-lysine - K(Ac))
  VARIANT 24: The peptide is substituted with an –NH2 group on its C-terminal extremity
LEGREXVRAXIXXEGXSTWSXRAX

SEQ ID NO: 44 - protein, 24 aa, Artificial Sequence
  Peptide analogue of the B-chain of Relaxin-2
  Peptide analogue of the B-chain of Relaxin-2
  VARIANT 1: The peptide is substituted with an acetyl (Ac) group on its N-terminal extremity
  VARIANT 10: Xaa in position 10 represents 2-amino-4-acetamido-hexanoic acid (Nε-Acetyl-lysine - K(Ac))
  VARIANT 12: Xaa in position 12 represents 2-amino-isobutyric acid (Aib)
  VARIANT 13: Xaa in position 13 represents 2-amino-isobutyric acid (Aib)
  VARIANT 16: Xaa in position 16 represents a lysine amino acid bound on the nitrogen atom of its lateral chain to a -(TTDS)3-(gamma glutamic acid)3-Palmitoyl group (-(TTDS)3-(gE)3-Palm)
  VARIANT 20: Xaa in position 20 represents D-serine (Dser)
  VARIANT 24: Xaa in position 24 represents 2-amino-4-acetamido-hexanoic acid (Nε-Acetyl-lysine - K(Ac))
  VARIANT 24: The peptide is substituted with an –NH2 group on its C-terminal extremity
LEGREKVRAXIXXEGXSTWXKRAX

SEQ ID NO: 45 - protein, 24 aa, Artificial Sequence
  Peptide analogue of the B-chain of Relaxin-2
  Peptide analogue of the B-chain of Relaxin-2
  VARIANT 1: The peptide is substituted with an acetyl (Ac) group on its N-terminal extremity
  VARIANT 10: Xaa in position 10 represents 2-amino-4-acetamido-hexanoic acid (Nε-Acetyl-lysine - K(Ac))
  VARIANT 12: Xaa in position 12 represents 2-amino-isobutyric acid (Aib)
  VARIANT 13: Xaa in position 13 represents 2-amino-isobutyric acid (Aib)
  VARIANT 16: Xaa in position 16 represents a lysine amino acid bound on the nitrogen atom of its lateral chain to a -(PEG2)5-(gamma glutamic acid)3-Palmitoyl group (-(PEG2)5-(gE)3-Palm)
  VARIANT 21: Xaa in position 21 represents α-Methyl-lysine (Mly)
  VARIANT 24: Xaa in position 24 represents 2-amino-4-acetamido-hexanoic acid (Nε-Acetyl-lysine - K(Ac))
  VARIANT 24: The peptide is substituted with an –NH2 group on its C-terminal extremity
LEGREKVRAXIXXEGXSTFSXRAX

SEQ ID NO: 46 - protein, 24 aa, Artificial Sequence
  Peptide analogue of the B-chain of Relaxin-2
  Peptide analogue of the B-chain of Relaxin-2
  VARIANT 1: The peptide is substituted with an acetyl (Ac) group on its N-terminal extremity
  VARIANT 10: Xaa in position 10 represents 2-amino-4-acetamido-hexanoic acid (Nε-Acetyl-lysine - K(Ac))
  VARIANT 12: Xaa in position 12 represents 2-amino-isobutyric acid (Aib)
  VARIANT 13: Xaa in position 13 represents 2-amino-isobutyric acid (Aib)
  VARIANT 16: Xaa in position 16 represents a lysine amino acid bound on the nitrogen atom of its lateral chain to a -(PEG2)5-(gamma glutamic acid)4-Palmitoyl group (-(PEG2)5-(gE)4-Palm)
  VARIANT 21: Xaa in position 21 represents α-Methyl-lysine (Mly)
  VARIANT 24: Xaa in position 24 represents 2-amino-4-acetamido-hexanoic acid (Nε-Acetyl-lysine - K(Ac))
  VARIANT 24: The peptide is substituted with an –NH2 group on its C-terminal extremity
LEGREKVRAXIXXEGXSTFSXRAX

SEQ ID NO: 47 - protein, 24 aa, Artificial Sequence
  Peptide analogue of the B-chain of Relaxin-2
  Peptide analogue of the B-chain of Relaxin-2
  VARIANT 1: The peptide is substituted with an acetyl (Ac) group on its N-terminal extremity
  VARIANT 12: Xaa in position 12 represents 2-amino-isobutyric acid (Aib)
  VARIANT 13: Xaa in position 13 represents 2-amino-isobutyric acid (Aib)
  VARIANT 16: Xaa in position 16 represents a lysine amino acid bound on the nitrogen atom of its lateral chain to a -(TTDS)3-(gamma glutamic acid)3-Palmitoyl group (-(TTDS)3-(gE)3-Palm)
  VARIANT 21: Xaa in position 21 represents α-Methyl-lysine (Mly)
  VARIANT 24: The peptide is substituted with an –NH2 group on its C-terminal extremity
  VARIANT 24: Xaa in position 24 represents 2-amino-4-acetamido-hexanoic acid (Nε-Acetyl-lysine - K(Ac))
LEGREKVRAKIXXEGXSTFSXRAX

SEQ ID NO: 48 - protein, 24 aa, Artificial Sequence
  Peptide analogue of the B-chain of Relaxin-2
  Peptide analogue of the B-chain of Relaxin-2
  VARIANT 1: The peptide is substituted with an acetyl (Ac) group on its N-terminal extremity
  VARIANT 12: Xaa in position 12 represents 2-amino-isobutyric acid (Aib)
  VARIANT 13: Xaa in position 13 represents 2-amino-isobutyric acid (Aib)
  VARIANT 16: Xaa in position 16 represents a lysine amino acid bound on the nitrogen atom of its lateral chain to a -(TTDS)3-(gamma glutamic acid)3-Palmitoyl group (-(TTDS)3-(gE)3-Palm)
  VARIANT 21: Xaa in position 21 represents α-Methyl-lysine (Mly)
  VARIANT 24: Xaa in position 24 represents 2-amino-4-acetamido-hexanoic acid (Nε-Acetyl-lysine - K(Ac))
  VARIANT 24: The peptide is substituted with an –NH2 group on its C-terminal extremity
LEGREKVRAQIXXEGXSTFSXRAX

SEQ ID NO: 49 - protein, 24 aa, Artificial Sequence
  Peptide analogue of the B-chain of Relaxin-2
  Peptide analogue of the B-chain of Relaxin-2
  VARIANT 1: The peptide is substituted with an acetyl (Ac) group on its N-terminal extremity
  VARIANT 10: Xaa in position 10 represents 2-amino-4-acetamido-hexanoic acid (Nε-Acetyl-lysine - K(Ac))
  VARIANT 12: Xaa in position 12 represents 2-amino-isobutyric acid (Aib)
  VARIANT 13: Xaa in position 13 represents 2-amino-isobutyric acid (Aib)
  VARIANT 16: Xaa in position 16 represents a lysine amino acid bound on the nitrogen atom of its lateral chain to a -(TTDS)3-(gamma glutamic acid)3-Palmitoyl group (-(TTDS)3-(gE)3-Palm)
  VARIANT 21: Xaa in position 21 represents α-Methyl-lysine (Mly)
  VARIANT 24: The peptide is substituted with an –NH2 group on its C-terminal extremity
LEGREKVRAXIXXEGXSTFSXRAK

SEQ ID NO: 50 - protein, 24 aa, Artificial Sequence
  Peptide analogue of the B-chain of Relaxin-2
  Peptide analogue of the B-chain of Relaxin-2
  VARIANT 1: The peptide is substituted with an acetyl (Ac) group on its N-terminal extremity
  VARIANT 10: Xaa in position 10 represents 2-amino-4-acetamido-hexanoic acid (Nε-Acetyl-lysine - K(Ac))
  VARIANT 12: Xaa in position 12 represents 2-amino-isobutyric acid (Aib)
  VARIANT 13: Xaa in position 13 represents 2-amino-isobutyric acid (Aib)
  VARIANT 16: Xaa in position 16 represents a lysine amino acid bound on the nitrogen atom of its lateral chain to a -(PEG2DGA)3-(gamma glutamic acid)3-Stearoyl group (-(PEG2DGA)3-(gE)3-Stea)
  VARIANT 21: Xaa in position 21 represents 2-amino-isobutyric acid (Aib)
  VARIANT 24: Xaa in position 24 represents 2-amino-4-acetamido-hexanoic acid (Nε-Acetyl-lysine - K(Ac))
  VARIANT 24: The peptide is substituted with an –NH2 group on its C-terminal extremity
LEGREKVRAXIXXEGXSTWSXRKX

SEQ ID NO: 51 - protein, 24 aa, Artificial Sequence
  Peptide analogue of the B-chain of Relaxin-2
  Peptide analogue of the B-chain of Relaxin-2
  VARIANT 1: The peptide is substituted with an acetyl (Ac) group on its N-terminal extremity
  VARIANT 10: Xaa in position 10 represents 2-amino-4-acetamido-hexanoic acid (Nε-Acetyl-lysine - K(Ac))
  VARIANT 12: Xaa in position 12 represents 2-amino-isobutyric acid (Aib)
  VARIANT 13: Xaa in position 13 represents 2-amino-isobutyric acid (Aib)
  VARIANT 16: Xaa in position 16 represents a lysine amino acid bound on the nitrogen atom of its lateral chain to a -(TTDS)3-(gamma glutamic acid)4-Stearoyl group (-(TTDS)3-(gE)4-Stea)
  VARIANT 21: Xaa in position 21 represents 2-amino-isobutyric acid (Aib)
  VARIANT 24: Xaa in position 24 represents 2-amino-4-acetamido-hexanoic acid (Nε-Acetyl-lysine - K(Ac))
  VARIANT 24: The peptide is substituted with an –NH2 group on its C-terminal extremity
LEGREKVRAXIXXEGXSTWSXRKX

SEQ ID NO: 52 - protein, 24 aa, Artificial Sequence
  Peptide analogue of the B-chain of Relaxin-2
  Peptide analogue of the B-chain of Relaxin-2
  VARIANT 1: The peptide is substituted with an acetyl (Ac) group on its N-terminal extremity
  VARIANT 10: Xaa in position 10 represents 2-amino-4-acetamido-hexanoic acid (Nε-Acetyl-lysine - K(Ac))
  VARIANT 12: Xaa in position 12 represents 2-amino-isobutyric acid (Aib)
  VARIANT 13: Xaa in position 13 represents 2-amino-isobutyric acid (Aib)
  VARIANT 16: Xaa in position 16 represents a lysine amino acid bound on the nitrogen atom of its lateral chain to a -(TTDS)3-(gamma glutamic acid)2-Stearoyl group (-(TTDS)3-(gE)2-Stea)
  VARIANT 21: Xaa in position 21 represents 2-amino-isobutyric acid (Aib)
  VARIANT 24: Xaa in position 24 represents 2-amino-4-acetamido-hexanoic acid (Nε-Acetyl-lysine - K(Ac))
  VARIANT 24: The peptide is substituted with an –NH2 group on its C-terminal extremity
LEGREKVRAXIXXEGXSTWSXRKX

SEQ ID NO: 53 - protein, 24 aa, Artificial Sequence
  Peptide analogue of the B-chain of Relaxin-2
  Peptide analogue of the B-chain of Relaxin-2
  VARIANT 1: The peptide is substituted with an acetyl (Ac) group on its N-terminal extremity
  VARIANT 10: Xaa in position 10 represents 2-amino-4-acetamido-hexanoic acid (Nε-Acetyl-lysine - K(Ac))
  VARIANT 12: Xaa in position 12 represents 2-amino-isobutyric acid (Aib)
  VARIANT 13: Xaa in position 13 represents 2-amino-isobutyric acid (Aib)
  VARIANT 16: Xaa in position 16 represents a lysine amino acid bound on the nitrogen atom of its lateral chain to a -(PEG2DGA)3-(gamma glutamic acid)4-Stearoyl group (-(PEG2DGA)3-(gE)4-Stea)
  VARIANT 21: Xaa in position 21 represents 2-amino-isobutyric acid (Aib)
  VARIANT 24: Xaa in position 24 represents 2-amino-4-acetamido-hexanoic acid (Nε-Acetyl-lysine - K(Ac))
  VARIANT 24: The peptide is substituted with an –NH2 group on its C-terminal extremity
LEGREKVRAXIXXEGXSTWSXRKX

SEQ ID NO: 54 - protein, 24 aa, Artificial Sequence
  Peptide analogue of the B-chain of Relaxin-2
  Peptide analogue of the B-chain of Relaxin-2
  VARIANT 1: The peptide is substituted with an acetyl (Ac) group on its N-terminal extremity
  VARIANT 10: Xaa in position 10 represents 2-amino-4-acetamido-hexanoic acid (Nε-Acetyl-lysine - K(Ac))
  VARIANT 12: Xaa in position 12 represents 2-amino-isobutyric acid (Aib)
  VARIANT 13: Xaa in position 13 represents 2-amino-isobutyric acid (Aib)
  VARIANT 16: Xaa in position 16 represents a lysine amino acid bound on the nitrogen atom of its lateral chain to a -(TTDS)2-(gamma glutamic acid)4-Stearoyl group (-(TTDS)2-(gE)4-Stea)
  VARIANT 21: Xaa in position 21 represents 2-amino-isobutyric acid (Aib)
  VARIANT 24: Xaa in position 24 represents 2-amino-4-acetamido-hexanoic acid (Nε-Acetyl-lysine - K(Ac))
  VARIANT 24: The peptide is substituted with an –NH2 group on its C-terminal extremity
LEGREKVRAXIXXEGXSTWSXRKX

SEQ ID NO: 55 - protein, 24 aa, Artificial Sequence
  Peptide analogue of the B-chain of Relaxin-2
  VARIANT 1: The peptide is substituted with an acetyl (Ac) group on its N-terminal extremity
  VARIANT 10: Xaa in position 10 represents 2-amino-4-acetamido-hexanoic acid (Nε-Acetyl-lysine - K(Ac))
  VARIANT 12: Xaa in position 12 represents 2-amino-isobutyric acid (Aib)
  VARIANT 13: Xaa in position 13 represents 2-amino-isobutyric acid (Aib)
  VARIANT 16: Xaa in position 16 represents a lysine amino acid bound on the nitrogen atom of its lateral chain to a -(TTDS)3-(gamma glutamic acid)3-Palmitoyl (-(TTDS)3-(gE)3-Palm)
  VARIANT 21: Xaa in position 21 represents 2-amino-isobutyric acid (Aib)
  VARIANT 24: The peptide is substituted with an –NH2 group on its C-terminal extremity
  VARIANT 24: Xaa in position 24 represents 2-amino-4-acetamido-hexanoic acid (Nε-Acetyl-lysine - K(Ac))
LEGRERVRAXIXXEGXSTWSXRRX

SEQ ID NO: 56 - protein, 24 aa, Artificial Sequence
  Peptide analogue of the B-chain of Relaxin-2
  VARIANT 1: The peptide is substituted with an acetyl (Ac) group on its N-terminal extremity
  VARIANT 10: Xaa in position 10 represents citruline (Cit)
  VARIANT 12: Xaa in position 12 represents 2-amino-isobutyric acid (Aib)
  VARIANT 13: Xaa in position 13 represents 2-amino-isobutyric acid (Aib)
  VARIANT 16: Xaa in position 16 represents a lysine amino acid bound on the nitrogen atom of its lateral chain to a -(TTDS)3-(gamma glutamic acid)3-Stearoyl (-(TTDS)3-(gE)3-Stea)
  VARIANT 21: Xaa in position 21 represents α-methyl-lysine (Mly)
  VARIANT 24: The peptide is substituted with an –NH2 group on its C-terminal extremity
  VARIANT 24: Xaa in position 24 represents 2-amino-4-acetamido-hexanoic acid (Nε-Acetyl-lysine - K(Ac))
LEGREKVRAXIXXEGXSTFSXRAX

SEQ ID NO: 57 - protein, 24 aa, Artificial Sequence
  Peptide analogue of the B-chain of Relaxin-2
  VARIANT 1: The peptide is substituted with an acetyl (Ac) group on its N-terminal extremity
  VARIANT 10: Xaa in position 10 represents 2-amino-4-acetamido-hexanoic acid (Nε-Acetyl-lysine - K(Ac))
  VARIANT 12: Xaa in position 12 represents 2-amino-isobutyric acid (Aib)
  VARIANT 13: Xaa in position 13 represents 2-amino-isobutyric acid (Aib)
  VARIANT 16: Xaa in position 16 represents a lysine amino acid bound on the nitrogen atom of its lateral chain to a -(TTDS)3-(gamma glutamic acid)3-Palmitoyl (-(TTDS)3-(gE)3-Palm)
  VARIANT 21: Xaa in position 21 represents homolysine (Hly)
  VARIANT 24: The peptide is substituted with an –NH2 group on its C-terminal extremity
  VARIANT 24: Xaa in position 24 represents 2-amino-4-acetamido-hexanoic acid (Nε-Acetyl-lysine - K(Ac))
LEGREKVRAXIXXEGXSTWSXRAX

SEQ ID NO: 58 - protein, 24 aa, Artificial Sequence
  Peptide analogue of the B-chain of Relaxin-2
  VARIANT 1: The peptide is substituted with an acetyl (Ac) group on its N-terminal extremity
  VARIANT 10: Xaa in position 10 represents 2-amino-4-acetamido-hexanoic acid (Nε-Acetyl-lysine - K(Ac))
  VARIANT 12: Xaa in position 12 represents 2-amino-isobutyric acid (Aib)
  VARIANT 13: Xaa in position 13 represents 2-amino-isobutyric acid (Aib)
  VARIANT 16: Xaa in position 16 represents a lysine amino acid bound on the nitrogen atom of its lateral chain to a -(TTDS)4-(gamma glutamic acid)3-Stearoyl (-(TTDS)4-(gE)3-Stea)
  VARIANT 21: Xaa in position 21 represents 2-amino-isobutyric acid (Aib)
  VARIANT 24: The peptide is substituted with an –NH2 group on its C-terminal extremity
  VARIANT 24: Xaa in position 24 represents 2-amino-4-acetamido-hexanoic acid (Nε-Acetyl-lysine - K(Ac))
LEGREKVRAXIXXEGXSTWSXRAX

SEQ ID NO: 59 - protein, 24 aa, Artificial Sequence
  Peptide analogue of the B-chain of Relaxin-2
  VARIANT 1: The peptide is substituted with an acetyl (Ac) group on its N-terminal extremity
  VARIANT 10: Xaa in position 10 represents 2-amino-4-acetamido-hexanoic acid (Nε-Acetyl-lysine - K(Ac))
  VARIANT 12: Xaa in position 12 represents 2-amino-isobutyric acid (Aib)
  VARIANT 13: Xaa in position 13 represents 2-amino-isobutyric acid (Aib)
  VARIANT 16: Xaa in position 16 represents a lysine amino acid bound on the nitrogen atom of its lateral chain to a -(TTDS)4-(gamma glutamic acid)3-Stearoyl (-(TTDS)4-(gE)3-Stea)
  VARIANT 21: Xaa in position 21 represents 2-amino-isobutyric acid (Aib)
  VARIANT 24: The peptide is substituted with an –NH2 group on its C-terminal extremity
  VARIANT 24: Xaa in position 24 represents 2-amino-4-acetamido-hexanoic acid (Nε-Acetyl-lysine - K(Ac))
LEGREKVRAXIXXEGXSTFSXRKX

SEQ ID NO: 60 - protein, 24 aa, Artificial Sequence
  Peptide analogue of the B-chain of Relaxin-2
  VARIANT 1: The peptide is substituted with an acetyl (Ac) group on its N-terminal extremity
  VARIANT 10: Xaa in position 10 represents 2-amino-4-acetamido-hexanoic acid (Nε-Acetyl-lysine - K(Ac))
  VARIANT 12: Xaa in position 12 represents 2-amino-isobutyric acid (Aib)
  VARIANT 13: Xaa in position 13 represents 2-amino-isobutyric acid (Aib)
  VARIANT 16: Xaa in position 16 represents a lysine amino acid bound on the nitrogen atom of its lateral chain to a -(TTDS)2-(gamma glutamic acid)3-Stearoyl (-(TTDS)2-(gE)3-Stea)
  VARIANT 21: Xaa in position 21 represents 2-amino-isobutyric acid (Aib)
  VARIANT 24: The peptide is substituted with an –NH2 group on its C-terminal extremity
  VARIANT 24: Xaa in position 24 represents 2-amino-4-acetamido-hexanoic acid (Nε-Acetyl-lysine - K(Ac))
LEGREKVRAXIXXEGXSTFSXRKX

SEQ ID NO: 61 - protein, 24 aa, Artificial Sequence
  Peptide analogue of the B-chain of Relaxin-2
  VARIANT 1: The peptide is substituted with an acetyl (Ac) group on its N-terminal extremity
  VARIANT 10: Xaa in position 10 represents 2-amino-4-acetamido-hexanoic acid (Nε-Acetyl-lysine - K(Ac))
  VARIANT 12: Xaa in position 12 represents 2-amino-isobutyric acid (Aib)
  VARIANT 13: Xaa in position 13 represents 2-amino-isobutyric acid (Aib)
  VARIANT 16: Xaa in position 16 represents a lysine amino acid bound on the nitrogen atom of its lateral chain to a -(TTDS)3-(gamma glutamic acid)3-Stearoyl (-(TTDS)3-(gE)3-Stea)
  VARIANT 21: Xaa in position 21 represents 2-amino-isobutyric acid (Aib)
  VARIANT 24: The peptide is substituted with an –NH2 group on its C-terminal extremity
  VARIANT 24: Xaa in position 24 represents 2-amino-4-acetamido-hexanoic acid (Nε-Acetyl-lysine - K(Ac))
LEGREKVRAXIXXEGXSTFSXRKX

SEQ ID NO: 62 - protein, 24 aa, Artificial Sequence
  Peptide analogue of the B-chain of Relaxin-2
  VARIANT 1: The peptide is substituted with an acetyl (Ac) group on its N-terminal extremity
  VARIANT 10: Xaa in position 10 represents 2-amino-4-acetamido-hexanoic acid (Nε-Acetyl-lysine - K(Ac))
  VARIANT 12: Xaa in position 12 represents 2-amino-isobutyric acid (Aib)
  VARIANT 13: Xaa in position 13 represents 2-amino-isobutyric acid (Aib)
  VARIANT 16: Xaa in position 16 represents a lysine amino acid bound on the nitrogen atom of its lateral chain to a -(TTDS)3-(gamma glutamic acid)4-Palmitoyl (-(TTDS)3-(gE)4-Palm)
  VARIANT 21: Xaa in position 21 represents 2-amino-isobutyric acid (Aib)
  VARIANT 24: The peptide is substituted with an –NH2 group on its C-terminal extremity
  VARIANT 24: Xaa in position 24 represents 2-amino-4-acetamido-hexanoic acid (Nε-Acetyl-lysine - K(Ac))
LEGREKVRAXIXXEGXSTWSXRKX

SEQ ID NO: 63 - protein, 24 aa, Artificial Sequence
  Peptide analogue of the B-chain of Relaxin-2
  VARIANT 1: The peptide is substituted with an acetyl (Ac) group on its N-terminal extremity
  VARIANT 10: Xaa in position 10 represents 2-amino-4-acetamido-hexanoic acid (Nε-Acetyl-lysine - K(Ac))
  VARIANT 12: Xaa in position 12 represents 2-amino-isobutyric acid (Aib)
  VARIANT 13: Xaa in position 13 represents 2-amino-isobutyric acid (Aib)
  VARIANT 16: Xaa in position 16 represents a lysine amino acid bound on the nitrogen atom of its lateral chain to a -(TTDS)3-(gamma glutamic acid)3-Palmitoyl (-(TTDS)3-(gE)3-Palm)
  VARIANT 21: Xaa in position 21 represents 2-amino-isobutyric acid (Aib)
  VARIANT 24: The peptide is substituted with an –NH2 group on its C-terminal extremity
  VARIANT 24: Xaa in position 24 represents 2-amino-4-acetamido-hexanoic acid (Nε-Acetyl-lysine - K(Ac))
LEGREKVRAXIXXEGXSQWSXRKX

SEQ ID NO: 64 - protein, 24 aa, Artificial Sequence
  Peptide analogue of the B-chain of Relaxin-2
  VARIANT 1: The peptide is substituted with an acetyl (Ac) group on its N-terminal extremity
  VARIANT 10: Xaa in position 10 represents 2-amino-4-acetamido-hexanoic acid (Nε-Acetyl-lysine - K(Ac))
  VARIANT 12: Xaa in position 12 represents 2-amino-isobutyric acid (Aib)
  VARIANT 13: Xaa in position 13 represents 2-amino-isobutyric acid (Aib)
  VARIANT 16: Xaa in position 16 represents a lysine amino acid bound on the nitrogen atom of its lateral chain to a -(TTDS)3-(gamma glutamic acid)3-Palmitoyl (-(TTDS)3-(gE)3-Palm)
  VARIANT 21: Xaa in position 21 represents 2-amino-isobutyric acid (Aib)
  VARIANT 24: The peptide is substituted with an –NH2 group on its C-terminal extremity
  VARIANT 24: Xaa in position 24 represents 2-amino-4-acetamido-hexanoic acid (Nε-Acetyl-lysine - K(Ac))
LEGREKVRAXIXXEGXSRWSXRKX

SEQ ID NO: 65 - protein, 24 aa, Artificial Sequence
  Peptide analogue of the B-chain of Relaxin-2
  VARIANT 1: The peptide is substituted with an acetyl (Ac) group on its N-terminal extremity
  VARIANT 9: Xaa in position 9 represents 2-amino-4-acetamido-hexanoic acid (Nε-Acetyl-lysine - K(Ac))
  VARIANT 12: Xaa in position 12 represents 2-amino-isobutyric acid (Aib)
  VARIANT 13: Xaa in position 13 represents 2-amino-isobutyric acid (Aib)
  VARIANT 16: Xaa in position 16 represents a lysine amino acid bound on the nitrogen atom of its lateral chain to a -(TTDS)3-(gamma glutamic acid)3-Palmitoyl (-(TTDS)3-(gE)3-Palm)
  VARIANT 21: Xaa in position 21 represents 2-amino-isobutyric acid (Aib)
  VARIANT 24: The peptide is substituted with an –NH2 group on its C-terminal extremity
  VARIANT 24: Xaa in position 24 represents 2-amino-4-acetamido-hexanoic acid (Nε-Acetyl-lysine - K(Ac))
LEGREKVRXQIXXEGXSTWSXRKX

SEQ ID NO: 66 - protein, 24 aa, Artificial Sequence
  Peptide analogue of the B-chain of Relaxin-2
  VARIANT 1: The peptide is substituted with an acetyl (Ac) group on its N-terminal extremity
  VARIANT 10: Xaa in position 10 represents 2-amino-4-acetamido-hexanoic acid (Nε-Acetyl-lysine - K(Ac))
  VARIANT 12: Xaa in position 12 represents 2-amino-isobutyric acid (Aib)
  VARIANT 13: Xaa in position 13 represents 2-amino-isobutyric acid (Aib)
  VARIANT 16: Xaa in position 16 represents a lysine amino acid bound on the nitrogen atom of its lateral chain to a -(TTDS)3-(gamma glutamic acid)3-Palmitoyl (-(TTDS)3-(gE)3-Palm)
  VARIANT 20: Xaa in position 20 represents 2-amino-4-acetamido-hexanoic acid (Nε-Acetyl-lysine - K(Ac))
  VARIANT 21: Xaa in position 21 represents 2-amino-isobutyric acid (Aib)
  VARIANT 24: The peptide is substituted with an –NH2 group on its C-terminal extremity
  VARIANT 24: Xaa in position 24 represents 2-amino-4-acetamido-hexanoic acid (Nε-Acetyl-lysine - K(Ac))
LEGREKVRAXIXXEGXSTWXXRAX

SEQ ID NO: 67 - protein, 24 aa, Artificial Sequence
  Peptide analogue of the B-chain of Relaxin-2
  VARIANT 1: The peptide is substituted with an acetyl (Ac) group on its N-terminal extremity
  VARIANT 10: Xaa in position 10 represents 2-amino-4-acetamido-hexanoic acid (Nε-Acetyl-lysine - K(Ac))
  VARIANT 12: Xaa in position 12 represents 2-amino-isobutyric acid (Aib)
  VARIANT 13: Xaa in position 13 represents 2-amino-isobutyric acid (Aib)
  VARIANT 16: Xaa in position 16 represents a lysine amino acid bound on the nitrogen atom of its lateral chain to a -(TTDS)3-(gamma glutamic acid)3-Palmitoyl (-(TTDS)3-(gE)3-Palm)
  VARIANT 21: Xaa in position 21 represents 2-amino-isobutyric acid (Aib)
  VARIANT 24: The peptide is substituted with an –NH2 group on its C-terminal extremity
  VARIANT 24: Xaa in position 24 represents 2-amino-4-acetamido-hexanoic acid (Nε-Acetyl-lysine - K(Ac))
LEGRERVRAXIXXEGXSTWSXRKX

SEQ ID NO: 68 - protein, 24 aa, Artificial Sequence
  Peptide analogue of the B-chain of Relaxin-2
  VARIANT 1: The peptide is substituted with an acetyl (Ac) group on its N-terminal extremity
  VARIANT 10: Xaa in position 10 represents 2-amino-4-acetamido-hexanoic acid (Nε-Acetyl-lysine - K(Ac))
  VARIANT 12: Xaa in position 12 represents 2-amino-isobutyric acid (Aib)
  VARIANT 13: Xaa in position 13 represents 2-amino-isobutyric acid (Aib)
  VARIANT 16: Xaa in position 16 represents a lysine amino acid bound on the nitrogen atom of its lateral chain to a -(TTDS)3-(gamma glutamic acid)3-Palmitoyl (-(TTDS)3-(gE)3-Palm)
  VARIANT 21: Xaa in position 21 represents 2-amino-isobutyric acid (Aib)
  VARIANT 23: Xaa in position 23 represents 2-amino-4-acetamido-hexanoic acid (Nε-Acetyl-lysine - K(Ac))
  VARIANT 24: The peptide is substituted with an –NH2 group on its C-terminal extremity
LEGREKVRAXIXXEGXSTWSXRXK

SEQ ID NO: 69 - protein, 24 aa, Artificial Sequence
  Peptide analogue of the B-chain of Relaxin-2
  VARIANT 1: The peptide is substituted with an acetyl (Ac) group on its N-terminal extremity
  VARIANT 10: Xaa in position 10 represents 2-amino-4-acetamido-hexanoic acid (Nε-Acetyl-lysine - K(Ac))
  VARIANT 12: Xaa in position 12 represents 2-amino-isobutyric acid (Aib)
  VARIANT 13: Xaa in position 13 represents 2-amino-isobutyric acid (Aib)
  VARIANT 16: Xaa in position 16 represents a lysine amino acid bound on the nitrogen atom of its lateral chain to a -(TTDS)3-(gamma glutamic acid)3-Palmitoyl (-(TTDS)3-(gE)3-Palm)
  VARIANT 21: Xaa in position 21 represents 2-amino-isobutyric acid (Aib)
  VARIANT 23: Xaa in position 23 represents 2-amino-4-acetamido-hexanoic acid (Nε-Acetyl-lysine - K(Ac))
  VARIANT 24: The peptide is substituted with an –NH2 group on its C-terminal extremity
LEGREKVRAXIXXEGXSTWSXRXR

SEQ ID NO: 70 - protein, 24 aa, Artificial Sequence
  Peptide analogue of the B-chain of Relaxin-2
  VARIANT 1: The peptide is substituted with an acetyl (Ac) group on its N-terminal extremity
  VARIANT 10: Xaa in position 10 represents 2-amino-4-acetamido-hexanoic acid (Nε-Acetyl-lysine - K(Ac))
  VARIANT 12: Xaa in position 12 represents 2-amino-isobutyric acid (Aib)
  VARIANT 16: Xaa in position 16 represents a lysine amino acid bound on the nitrogen atom of its lateral chain to a -(TTDS)3-(gamma glutamic acid)3-Palmitoyl (-(TTDS)3-(gE)3-Palm)
  VARIANT 21: Xaa in position 21 represents 2-amino-isobutyric acid (Aib)
  VARIANT 24: The peptide is substituted with an –NH2 group on its C-terminal extremity
  VARIANT 24: Xaa in position 24 represents 2-amino-4-acetamido-hexanoic acid (Nε-Acetyl-lysine - K(Ac))
LEGREKVRAXIXIEGXSTWSXRKX

SEQ ID NO: 71 - protein, 24 aa, Artificial Sequence
  Peptide analogue of the B-chain of Relaxin-2
  VARIANT 1: The peptide is substituted with an acetyl (Ac) group on its N-terminal extremity
  VARIANT 10: Xaa in position 10 represents 2-amino-4-acetamido-hexanoic acid (Nε-Acetyl-lysine - K(Ac))
  VARIANT 12: Xaa in position 12 represents 2-amino-isobutyric acid (Aib)
  VARIANT 13: Xaa in position 13 represents 2-amino-isobutyric acid (Aib)
  VARIANT 16: Xaa in position 16 represents a lysine amino acid bound on the nitrogen atom of its lateral chain to a -(TTDS)3-(gamma glutamic acid)3-Palmitoyl (-(TTDS)3-(gE)3-Palm)
  VARIANT 21: Xaa in position 21 represents 2-amino-isobutyric acid (Aib)
  VARIANT 24: The peptide is substituted with an –NH2 group on its C-terminal extremity
LEGREKVRAXIXXEGXSTWSXRAK

SEQ ID NO: 72 - protein, 24 aa, Artificial Sequence
  Peptide analogue of the B-chain of Relaxin-2
  VARIANT 1: The peptide is substituted with an acetyl (Ac) group on its N-terminal extremity
  VARIANT 10: Xaa in position 10 represents 2-amino-4-acetamido-hexanoic acid (Nε-Acetyl-lysine - K(Ac))
  VARIANT 12: Xaa in position 12 represents 2-amino-isobutyric acid (Aib)
  VARIANT 13: Xaa in position 13 represents 2-amino-isobutyric acid (Aib)
  VARIANT 16: Xaa in position 16 represents a lysine amino acid bound on the nitrogen atom of its lateral chain to a -(TTDS)3-(gamma glutamic acid)3-Palmitoyl (-(TTDS)3-(gE)3-Palm)
  VARIANT 20: Xaa in position 20 represents 2-amino-isobutyric acid (Aib)
  VARIANT 24: The peptide is substituted with an –NH2 group on its C-terminal extremity
  VARIANT 24: Xaa in position 24 represents 2-amino-4-acetamido-hexanoic acid (Nε-Acetyl-lysine - K(Ac))
LEGREKVRAXIXXEGXSTFXRRAX

SEQ ID NO: 73 - protein, 24 aa, Artificial Sequence
  Peptide analogue of the B-chain of Relaxin-2
  VARIANT 1: The peptide is substituted with an acetyl (Ac) group on its N-terminal extremity
  VARIANT 10: Xaa in position 10 represents 2-amino-4-acetamido-hexanoic acid (Nε-Acetyl-lysine - K(Ac))
  VARIANT 12: Xaa in position 12 represents 2-amino-isobutyric acid (Aib)
  VARIANT 13: Xaa in position 13 represents 2-amino-isobutyric acid (Aib)
  VARIANT 16: Xaa in position 16 represents a lysine amino acid bound on the nitrogen atom of its lateral chain to a -(TTDS)3-(gamma glutamic acid)3-Palmitoyl (-(TTDS)3-(gE)3-Palm)
  VARIANT 21: Xaa in position 21 represents 2-amino-isobutyric acid (Aib)
  VARIANT 24: The peptide is substituted with an –NH2 group on its C-terminal extremity
LEGREKVRAXIXXEGXSKWSXRAK

SEQ ID NO: 74 - protein, 24 aa, Artificial Sequence
  Peptide analogue of the B-chain of Relaxin-2
  VARIANT 1: The peptide is substituted with an acetyl (Ac) group on its N-terminal extremity
  VARIANT 10: Xaa in position 10 represents 2-amino-4-acetamido-hexanoic acid (Nε-Acetyl-lysine - K(Ac))
  VARIANT 12: Xaa in position 12 represents 2-amino-isobutyric acid (Aib)
  VARIANT 16: Xaa in position 16 represents a lysine amino acid bound on the nitrogen atom of its lateral chain to a -(TTDS)4-(gamma glutamic acid)3-Palmitoyl (-(TTDS)4-(gE)3-Palm)
  VARIANT 21: Xaa in position 21 represents 2-amino-isobutyric acid (Aib)
  VARIANT 24: The peptide is substituted with an –NH2 group on its C-terminal extremity
  VARIANT 24: Xaa in position 24 represents 2-amino-4-acetamido-hexanoic acid (Nε-Acetyl-lysine - K(Ac))
LEGREKVRAXIXIEGXSTWSXRKX

SEQ ID NO: 75 - protein, 24 aa, Artificial Sequence
  Peptide analogue of the B-chain of Relaxin-2
  VARIANT 1: The peptide is substituted with an acetyl (Ac) group on its N-terminal extremity
  VARIANT 10: Xaa in position 10 represents 2-amino-4-acetamido-hexanoic acid (Nε-Acetyl-lysine - K(Ac))
  VARIANT 12: Xaa in position 12 represents 2-amino-isobutyric acid (Aib)
  VARIANT 13: Xaa in position 13 represents 2-amino-isobutyric acid (Aib)
  VARIANT 16: Xaa in position 16 represents a lysine amino acid bound on the nitrogen atom of its lateral chain to a -(TTDS)4-(gamma glutamic acid)3-Palmitoyl (-(TTDS)4-(gE)3-Palm)
  VARIANT 21: Xaa in position 21 represents 2-amino-isobutyric acid (Aib)
  VARIANT 24: The peptide is substituted with an –NH2 group on its C-terminal extremity
  VARIANT 24: Xaa in position 24 represents 2-amino-4-acetamido-hexanoic acid (Nε-Acetyl-lysine - K(Ac))
LEGRERVRAXIXXEGXSTWSXRRX

SEQ ID NO: 76 - protein, 24 aa, Artificial Sequence
  Peptide analogue of the B-chain of Relaxin-2
  VARIANT 1: The peptide is substituted with an acetyl (Ac) group on its N-terminal extremity
  VARIANT 10: Xaa in position 10 represents 2-amino-4-acetamido-hexanoic acid (Nε-Acetyl-lysine - K(Ac))
  VARIANT 12: Xaa in position 12 represents 2-amino-isobutyric acid (Aib)
  VARIANT 13: Xaa in position 13 represents 2-amino-isobutyric acid (Aib)
  VARIANT 16: Xaa in position 16 represents a lysine amino acid bound on the nitrogen atom of its lateral chain to a -(TTDS)3-(gamma glutamic acid)3-Palmitoyl (-(TTDS)3-(gE)3-Palm)
  VARIANT 21: Xaa in position 21 represents 2-amino-isobutyric acid (Aib)
  VARIANT 24: The peptide is substituted with an –NH2 group on its C-terminal extremity
  VARIANT 24: Xaa in position 24 represents 2-amino-4-acetamido-hexanoic acid (Nε-Acetyl-lysine - K(Ac))
LEGRERVRAXIXXEGXSTFSXRRX

SEQ ID NO: 77 - protein, 24 aa, Artificial Sequence
  Peptide analogue of the B-chain of Relaxin-2
  VARIANT 1: The peptide is substituted with an acetyl (Ac) group on its N-terminal extremity
  VARIANT 10: Xaa in position 10 represents 2-amino-4-acetamido-hexanoic acid (Nε-Acetyl-lysine - K(Ac))
  VARIANT 12: Xaa in position 12 represents 2-amino-isobutyric acid (Aib)
  VARIANT 13: Xaa in position 13 represents 2-amino-isobutyric acid (Aib)
  VARIANT 16: Xaa in position 16 represents a lysine amino acid bound on the nitrogen atom of its lateral chain to a -(TTDS)4-(gamma glutamic acid)3-Palmitoyl (-(TTDS)4-(gE)3-Palm)
  VARIANT 21: Xaa in position 21 represents 2-amino-isobutyric acid (Aib)
  VARIANT 24: The peptide is substituted with an –NH2 group on its C-terminal extremity
  VARIANT 24: Xaa in position 24 represents 2-amino-4-acetamido-hexanoic acid (Nε-Acetyl-lysine - K(Ac))
LEGRERVRAXIXXEGXSTFSXRRX

SEQ ID NO: 78 - protein, 24 aa, Artificial Sequence
  Peptide analogue of the B-chain of Relaxin-2
  VARIANT 1: The peptide is substituted with an acetyl (Ac) group on its N-terminal extremity
  VARIANT 10: Xaa in position 10 represents 2-amino-4-acetamido-hexanoic acid (Nε-Acetyl-lysine - K(Ac))
  VARIANT 12: Xaa in position 12 represents 2-amino-isobutyric acid (Aib)
  VARIANT 13: Xaa in position 13 represents 2-amino-isobutyric acid (Aib)
  VARIANT 16: Xaa in position 16 represents a lysine amino acid bound on the nitrogen atom of its lateral chain to a -(TTDS)4-(gamma glutamic acid)3-Palmitoyl (-(TTDS)4-(gE)3-Palm)
  VARIANT 21: Xaa in position 21 represents α-methyl-lysine (Mly)
  VARIANT 24: The peptide is substituted with an –NH2 group on its C-terminal extremity
  VARIANT 24: Xaa in position 24 represents 2-amino-4-acetamido-hexanoic acid (Nε-Acetyl-lysine - K(Ac))
LEGREKVRAXIXXEGXSTFSXRAX

SEQ ID NO: 79 - protein, 24 aa, Artificial Sequence
  Peptide analogue of the B-chain of Relaxin-2
  VARIANT 1: The peptide is substituted with an acetyl (Ac) group on its N-terminal extremity
  VARIANT 10: Xaa in position 10 represents 2-amino-4-acetamido-hexanoic acid (Nε-Acetyl-lysine - K(Ac))
  VARIANT 12: Xaa in position 12 represents 2-amino-isobutyric acid (Aib)
  VARIANT 13: Xaa in position 13 represents 2-amino-isobutyric acid (Aib)
  VARIANT 16: Xaa in position 16 represents a lysine amino acid bound on the nitrogen atom of its lateral chain to a -(TTDS)3-(gamma glutamic acid)3-Palmitoyl (-(TTDS)3-(gE)3-Palm)
  VARIANT 21: Xaa in position 21 represents 2-amino-isobutyric acid (Aib)
  VARIANT 24: The peptide is substituted with an –NH2 group on its C-terminal extremity
  VARIANT 24: Xaa in position 24 represents 2-amino-4-acetamido-hexanoic acid (Nε-Acetyl-lysine - K(Ac))
LEGREKVRAXIXXEGXSKFSXRKX

SEQ ID NO: 80 - protein, 24 aa, Artificial Sequence
  Peptide analogue of the B-chain of Relaxin-2
  VARIANT 1: The peptide is substituted with an acetyl (Ac) group on its N-terminal extremity
  VARIANT 10: Xaa in position 10 represents 2-amino-4-acetamido-hexanoic acid (Nε-Acetyl-lysine - K(Ac))
  VARIANT 12: Xaa in position 12 represents 2-amino-isobutyric acid (Aib)
  VARIANT 13: Xaa in position 13 represents 2-amino-isobutyric acid (Aib)
  VARIANT 16: Xaa in position 16 represents a lysine amino acid bound on the nitrogen atom of its lateral chain to a -(TTDS)3-(gamma glutamic acid)3-Palmitoyl (-(TTDS)3-(gE)3-Palm)
  VARIANT 19: Xaa in position 19 represents 5-chloro-tryptophan (Trp(5Cl))
  VARIANT 21: Xaa in position 21 represents 2-amino-isobutyric acid (Aib)
  VARIANT 24: The peptide is substituted with an –NH2 group on its C-terminal extremity
  VARIANT 24: Xaa in position 24 represents 2-amino-4-acetamido-hexanoic acid (Nε-Acetyl-lysine - K(Ac))
LEGRERVRAXIXXEGXSTXSXRRX

SEQ ID NO: 81 - protein, 24 aa, Artificial Sequence
  Peptide analogue of the B-chain of Relaxin-2
  VARIANT 1: The peptide is substituted with an acetyl (Ac) group on its N-terminal extremity
  VARIANT 1: Xaa in position 1 represents 2-amino-4-acetamido-hexanoic acid (Nε-Acetyl-lysine - K(Ac))
  VARIANT 10: Xaa in position 10 represents 2-amino-4-acetamido-hexanoic acid (Nε-Acetyl-lysine - K(Ac))
  VARIANT 12: Xaa in position 12 represents 2-amino-isobutyric acid (Aib)
  VARIANT 13: Xaa in position 13 represents 2-amino-isobutyric acid (Aib)
  VARIANT 16: Xaa in position 16 represents a lysine amino acid bound on the nitrogen atom of its lateral chain to a -(TTDS)3-(gamma glutamic acid)3-Palmitoyl (-(TTDS)3-(gE)3-Palm)
  VARIANT 21: Xaa in position 21 represents α-methyl-lysine (Mly)
  VARIANT 24: The peptide is substituted with an –NH2 group on its C-terminal extremity
  VARIANT 24: Xaa in position 24 represents 2-amino-4-acetamido-hexanoic acid (Nε-Acetyl-lysine - K(Ac))
XEGREKVRAXIXXEGXSTFSXRAX

SEQ ID NO: 82 - protein, 24 aa, Artificial Sequence
  Peptide analogue of the B-chain of Relaxin-2
  VARIANT 1: The peptide is substituted with an acetyl (Ac) group on its N-terminal extremity
  VARIANT 9: Xaa in position 9 represents 2-amino-isobutyric acid (Aib)
  VARIANT 10: Xaa in position 10 represents 2-amino-4-acetamido-hexanoic acid (Nε-Acetyl-lysine - K(Ac))
  VARIANT 12: Xaa in position 12 represents 2-amino-isobutyric acid (Aib)
  VARIANT 13: Xaa in position 13 represents 2-amino-isobutyric acid (Aib)
  VARIANT 16: Xaa in position 16 represents a lysine amino acid bound on the nitrogen atom of its lateral chain to a -(TTDS)3-(gamma glutamic acid)3-Palmitoyl (-(TTDS)3-(gE)3-Palm)
  VARIANT 21: Xaa in position 21 represents 2-amino-isobutyric acid (Aib)
  VARIANT 24: The peptide is substituted with an –NH2 group on its C-terminal extremity
  VARIANT 24: Xaa in position 24 represents 2-amino-4-acetamido-hexanoic acid (Nε-Acetyl-lysine - K(Ac))
LEGREKVRXXIXXEGXSTWSXRAX

SEQ ID NO: 83 - protein, 24 aa, Artificial Sequence
  Peptide analogue of the B-chain of Relaxin-2
  VARIANT 1: The peptide is substituted with an acetyl (Ac) group on its N-terminal extremity
  VARIANT 10: Xaa in position 10 represents 2-amino-4-acetamido-hexanoic acid (Nε-Acetyl-lysine - K(Ac))
  VARIANT 12: Xaa in position 12 represents 2-amino-isobutyric acid (Aib)
  VARIANT 13: Xaa in position 13 represents 2-amino-isobutyric acid (Aib)
  VARIANT 16: Xaa in position 16 represents a lysine amino acid bound on the nitrogen atom of its lateral chain to a -(TTDS)3-(gamma glutamic acid)3-Palmitoyl (-(TTDS)3-(gE)3-Palm)
  VARIANT 21: Xaa in position 21 represents 2-amino-isobutyric acid (Aib)
  VARIANT 24: The peptide is substituted with an –NH2 group on its C-terminal extremity
  VARIANT 24: Xaa in position 24 represents 2-amino-4-acetamido-hexanoic acid (Nε-Acetyl-lysine - K(Ac))
LEGREKVRAXIXXEGXSKWSXRKX

SEQ ID NO: 84 - protein, 24 aa, Artificial Sequence
  Peptide analogue of the B-chain of Relaxin-2
  VARIANT 1: The peptide is substituted with an acetyl (Ac) group on its N-terminal extremity
  VARIANT 10: Xaa in position 10 represents 2-amino-4-acetamido-hexanoic acid (Nε-Acetyl-lysine - K(Ac))
  VARIANT 12: Xaa in position 12 represents 2-amino-isobutyric acid (Aib)
  VARIANT 16: Xaa in position 16 represents a lysine amino acid bound on the nitrogen atom of its lateral chain to a -(TTDS)3-(gamma glutamic acid)3-Palmitoyl (-(TTDS)3-(gE)3-Palm)
  VARIANT 21: Xaa in position 21 represents α-methyl-lysine (Mly)
  VARIANT 24: The peptide is substituted with an –NH2 group on its C-terminal extremity
  VARIANT 24: Xaa in position 24 represents 2-amino-4-acetamido-hexanoic acid (Nε-Acetyl-lysine - K(Ac))
LEGREKVRAXIXIEGXSTFSXRAX

SEQ ID NO: 85 - protein, 24 aa, Artificial Sequence
  Peptide analogue of the B-chain of Relaxin-2
  VARIANT 1: The peptide is substituted with an acetyl (Ac) group on its N-terminal extremity
  VARIANT 9: Xaa in position 9 represents 2-amino-isobutyric acid (Aib)
  VARIANT 10: Xaa in position 10 represents 2-amino-4-acetamido-hexanoic acid (Nε-Acetyl-lysine - K(Ac))
  VARIANT 12: Xaa in position 12 represents 2-amino-isobutyric acid (Aib)
  VARIANT 13: Xaa in position 13 represents 2-amino-isobutyric acid (Aib)
  VARIANT 16: Xaa in position 16 represents a lysine amino acid bound on the nitrogen atom of its lateral chain to a -(TTDS)3-(gamma glutamic acid)3-Palmitoyl (-(TTDS)3-(gE)3-Palm)
  VARIANT 21: Xaa in position 21 represents 2-amino-isobutyric acid (Aib)
  VARIANT 24: The peptide is substituted with an –NH2 group on its C-terminal extremity
  VARIANT 24: Xaa in position 24 represents 2-amino-4-acetamido-hexanoic acid (Nε-Acetyl-lysine - K(Ac))
LEGRERVRXXIXXEGXSTWSXRRX

SEQ ID NO: 86 - protein, 24 aa, Artificial Sequence
  Peptide analogue of the B-chain of Relaxin-2
  VARIANT 1: The peptide is substituted with an acetyl (Ac) group on its N-terminal extremity
  VARIANT 1: Xaa in position 1 represents 2-amino-isobutyric acid (Aib)
  VARIANT 10: Xaa in position 10 represents 2-amino-4-acetamido-hexanoic acid (Nε-Acetyl-lysine - K(Ac))
  VARIANT 12: Xaa in position 12 represents 2-amino-isobutyric acid (Aib)
  VARIANT 16: Xaa in position 16 represents a lysine amino acid bound on the nitrogen atom of its lateral chain to a -(TTDS)3-(gamma glutamic acid)3-Palmitoyl (-(TTDS)3-(gE)3-Palm)
  VARIANT 21: Xaa in position 21 represents α-methyl-lysine (Mly)
  VARIANT 24: The peptide is substituted with an –NH2 group on its C-terminal extremity
  VARIANT 24: Xaa in position 24 represents 2-amino-4-acetamido-hexanoic acid (Nε-Acetyl-lysine - K(Ac))
XEGREKVRAXIXIEGXSTFSXRAX

SEQ ID NO: 87 - protein, 24 aa, Artificial Sequence
  Peptide analogue of the B-chain of Relaxin-2
  VARIANT 1: The peptide is substituted with an acetyl (Ac) group on its N-terminal extremity
  VARIANT 10: Xaa in position 10 represents 2-amino-4-acetamido-hexanoic acid (Nε-Acetyl-lysine - K(Ac))
  VARIANT 12: Xaa in position 12 represents 2-amino-isobutyric acid (Aib)
  VARIANT 13: Xaa in position 13 represents 2-amino-isobutyric acid (Aib)
  VARIANT 16: Xaa in position 16 represents a lysine amino acid bound on the nitrogen atom of its lateral chain to a -(TTDS)3-(gamma glutamic acid)3-Palmitoyl (-(TTDS)3-(gE)3-Palm)
  VARIANT 24: The peptide is substituted with an –NH2 group on its C-terminal extremity
  VARIANT 24: Xaa in position 24 represents 2-amino-4-acetamido-hexanoic acid (Nε-Acetyl-lysine - K(Ac))
LEGREKVRAXIXXEGXSTFSRRAX

SEQ ID NO: 88 - protein, 24 aa, Artificial Sequence
  Peptide analogue of the B-chain of Relaxin-2
  VARIANT 1: The peptide is substituted with an acetyl (Ac) group on its N-terminal extremity
  VARIANT 10: Xaa in position 10 represents 2-amino-4-acetamido-hexanoic acid (Nε-Acetyl-lysine - K(Ac))
  VARIANT 12: Xaa in position 12 represents 2-amino-isobutyric acid (Aib)
  VARIANT 13: Xaa in position 13 represents 2-amino-isobutyric acid (Aib)
  VARIANT 16: Xaa in position 16 represents a lysine amino acid bound on the nitrogen atom of its lateral chain to a -(TTDS)3-(gamma glutamic acid)3-Palmitoyl (-(TTDS)3-(gE)3-Palm)
  VARIANT 21: Xaa in position 21 represents homolysine (Hly)
  VARIANT 24: The peptide is substituted with an –NH2 group on its C-terminal extremity
  VARIANT 24: Xaa in position 24 represents 2-amino-4-acetamido-hexanoic acid (Nε-Acetyl-lysine - K(Ac))
LEGREKVRAXIXXEGXSTFSXRAX

SEQ ID NO: 89 - protein, 24 aa, Artificial Sequence
  Peptide analogue of the B-chain of Relaxin-2
  VARIANT 1: The peptide is substituted with an acetyl (Ac) group on its N-terminal extremity
  VARIANT 10: Xaa in position 10 represents 2-amino-4-acetamido-hexanoic acid (Nε-Acetyl-lysine - K(Ac))
  VARIANT 12: Xaa in position 12 represents 2-amino-isobutyric acid (Aib)
  VARIANT 13: Xaa in position 13 represents 2-amino-isobutyric acid (Aib)
  VARIANT 16: Xaa in position 16 represents a lysine amino acid bound on the nitrogen atom of its lateral chain to a -(TTDS)3-(gamma glutamic acid)3-Palmitoyl (-(TTDS)3-(gE)3-Palm)
  VARIANT 19: Xaa in position 19 represents α-methyl-phenylalanine (Mph)
  VARIANT 24: The peptide is substituted with an –NH2 group on its C-terminal extremity
  VARIANT 24: Xaa in position 24 represents 2-amino-4-acetamido-hexanoic acid (Nε-Acetyl-lysine - K(Ac))
LEGREKVRAXIXXEGXSTXSRRAX

SEQ ID NO: 90 - protein, 24 aa, Artificial Sequence
  Peptide analogue of the B-chain of Relaxin-2
  VARIANT 1: The peptide is substituted with an acetyl (Ac) group on its N-terminal extremity
  VARIANT 10: Xaa in position 10 represents 2-amino-4-acetamido-hexanoic acid (Nε-Acetyl-lysine - K(Ac))
  VARIANT 13: Xaa in position 13 represents 2-amino-isobutyric acid (Aib)
  VARIANT 16: Xaa in position 16 represents a lysine amino acid bound on the nitrogen atom of its lateral chain to a -(TTDS)3-(gamma glutamic acid)3-Palmitoyl (-(TTDS)3-(gE)3-Palm)
  VARIANT 21: Xaa in position 21 represents α-methyl-lysine (Mly)
  VARIANT 24: The peptide is substituted with an –NH2 group on its C-terminal extremity
  VARIANT 24: Xaa in position 24 represents 2-amino-4-acetamido-hexanoic acid (Nε-Acetyl-lysine - K(Ac))
LEGREKVRAXIAXEGXSTFSXRAX

SEQ ID NO: 91 - protein, 24 aa, Artificial Sequence
  Peptide analogue of the B-chain of Relaxin-2
  VARIANT 1: The peptide is substituted with an acetyl (Ac) group on its N-terminal extremity
  VARIANT 10: Xaa in position 10 represents 2-amino-4-acetamido-hexanoic acid (Nε-Acetyl-lysine - K(Ac))
  VARIANT 12: Xaa in position 12 represents 2-amino-isobutyric acid (Aib)
  VARIANT 13: Xaa in position 13 represents 2-amino-isobutyric acid (Aib)
  VARIANT 16: Xaa in position 16 represents a lysine amino acid bound on the nitrogen atom of its lateral chain to a -(TTDS)3-(gamma glutamic acid)3-Palmitoyl (-(TTDS)3-(gE)3-Palm)
  VARIANT 19: Xaa in position 19 represents 4-fluoro-phenylalanine (Pfp)
  VARIANT 21: Xaa in position 21 represents 2-amino-isobutyric acid (Aib)
  VARIANT 24: The peptide is substituted with an –NH2 group on its C-terminal extremity
  VARIANT 24: Xaa in position 24 represents 2-amino-4-acetamido-hexanoic acid (Nε-Acetyl-lysine - K(Ac))
LEGRERVRAXIXXEGXSTXSXRRX

SEQ ID NO: 92 - protein, 24 aa, Artificial Sequence
  Peptide analogue of the B-chain of Relaxin-2
  VARIANT 1: The peptide is substituted with an acetyl (Ac) group on its N-terminal extremity
  VARIANT 10: Xaa in position 10 represents 2-amino-4-acetamido-hexanoic acid (Nε-Acetyl-lysine - K(Ac))
  VARIANT 12: Xaa in position 12 represents 2-amino-isobutyric acid (Aib)
  VARIANT 13: Xaa in position 13 represents 2-amino-isobutyric acid (Aib)
  VARIANT 16: Xaa in position 16 represents a lysine amino acid bound on the nitrogen atom of its lateral chain to a -(TTDS)3-(gamma glutamic acid)3-Palmitoyl (-(TTDS)3-(gE)3-Palm)
  VARIANT 19: Xaa in position 19 represents 5-fluoro-tryptophan (Trp(5F))
  VARIANT 21: Xaa in position 21 represents 2-amino-isobutyric acid (Aib)
  VARIANT 24: The peptide is substituted with an –NH2 group on its C-terminal extremity
  VARIANT 24: Xaa in position 24 represents 2-amino-4-acetamido-hexanoic acid (Nε-Acetyl-lysine - K(Ac))
LEGRERVRAXIXXEGXSTXSXRRX

SEQ ID NO: 93 - protein, 24 aa, Artificial Sequence
  Peptide analogue of the B-chain of Relaxin-2
  VARIANT 1: The peptide is substituted with an acetyl (Ac) group on its N-terminal extremity
  VARIANT 10: Xaa in position 10 represents 2-amino-4-acetamido-hexanoic acid (Nε-Acetyl-lysine - K(Ac))
  VARIANT 12: Xaa in position 12 represents 2-amino-isobutyric acid (Aib)
  VARIANT 13: Xaa in position 13 represents 2-amino-isobutyric acid (Aib)
  VARIANT 16: Xaa in position 16 represents a lysine amino acid bound on the nitrogen atom of its lateral chain to a -(TTDS)3-(gamma glutamic acid)3-Palmitoyl (-(TTDS)3-(gE)3-Palm)
  VARIANT 24: The peptide is substituted with an –NH2 group on its C-terminal extremity
  VARIANT 24: Xaa in position 24 represents 2-amino-4-acetamido-hexanoic acid (Nε-Acetyl-lysine - K(Ac))
LEGREKVRAXIXXEGXSTFTRRAX

SEQ ID NO: 94 - protein, 24 aa, Artificial Sequence
  Peptide analogue of the B-chain of Relaxin-2
  VARIANT 1: The peptide is substituted with an acetyl (Ac) group on its N-terminal extremity
  VARIANT 10: Xaa in position 10 represents 2-amino-4-acetamido-hexanoic acid (Nε-Acetyl-lysine - K(Ac))
  VARIANT 12: Xaa in position 12 represents 2-amino-isobutyric acid (Aib)
  VARIANT 13: Xaa in position 13 represents 2-amino-isobutyric acid (Aib)
  VARIANT 16: Xaa in position 16 represents a lysine amino acid bound on the nitrogen atom of its lateral chain to a -(TTDS)3-(gamma glutamic acid)3-Palmitoyl (-(TTDS)3-(gE)3-Palm)
  VARIANT 24: The peptide is substituted with an –NH2 group on its C-terminal extremity
  VARIANT 24: Xaa in position 24 represents 2-amino-4-acetamido-hexanoic acid (Nε-Acetyl-lysine - K(Ac))
LEGREKVRAXIXXEGXSTFVRRAX

SEQ ID NO: 95 - protein, 24 aa, Artificial Sequence
  Peptide analogue of the B-chain of Relaxin-2
  VARIANT 1: The peptide is substituted with an acetyl (Ac) group on its N-terminal extremity
  VARIANT 10: Xaa in position 10 represents 2-amino-4-acetamido-hexanoic acid (Nε-Acetyl-lysine - K(Ac))
  VARIANT 12: Xaa in position 12 represents 2-amino-isobutyric acid (Aib)
  VARIANT 13: Xaa in position 13 represents 2-amino-isobutyric acid (Aib)
  VARIANT 16: Xaa in position 16 represents a lysine amino acid bound on the nitrogen atom of its lateral chain to a -(TTDS)3-(gamma glutamic acid)3-Myristoyl (-(TTDS)3-(gE)3-Myr)
  VARIANT 21: Xaa in position 21 represents α-methyl-lysine (Mly)
  VARIANT 24: The peptide is substituted with an –NH2 group on its C-terminal extremity
  VARIANT 24: Xaa in position 24 represents 2-amino-4-acetamido-hexanoic acid (Nε-Acetyl-lysine - K(Ac))
LEGREKVRAXIXXEGXSTFSXRAX

SEQ ID NO: 96 - protein, 24 aa, Artificial Sequence
  Peptide analogue of the B-chain of Relaxin-2
  VARIANT 1: The peptide is substituted with an acetyl (Ac) group on its N-terminal extremity
  VARIANT 10: Xaa in position 10 represents 2-amino-4-acetamido-hexanoic acid (Nε-Acetyl-lysine - K(Ac))
  VARIANT 12: Xaa in position 12 represents 2-amino-isobutyric acid (Aib)
  VARIANT 13: Xaa in position 13 represents 2-amino-isobutyric acid (Aib)
  VARIANT 16: Xaa in position 16 represents a lysine amino acid bound on the nitrogen atom of its lateral chain to a -(TTDS)3-(gamma glutamic acid)3-Myristoyl (-(TTDS)3-(gE)3-Myr)
  VARIANT 21: Xaa in position 21 represents α-methyl-lysine (Mly)
  VARIANT 24: The peptide is substituted with an –NH2 group on its C-terminal extremity
LEGREKVRAXIXXEGXSTFSXRAK

SEQ ID NO: 97 - protein, 24 aa, Artificial Sequence
  Peptide analogue of the B-chain of Relaxin-2
  VARIANT 1: The peptide is substituted with an acetyl (Ac) group on its N-terminal extremity
  VARIANT 10: Xaa in position 10 represents 2-amino-4-acetamido-hexanoic acid (Nε-Acetyl-lysine - K(Ac))
  VARIANT 12: Xaa in position 12 represents 2-amino-isobutyric acid (Aib)
  VARIANT 13: Xaa in position 13 represents 2-amino-isobutyric acid (Aib)
  VARIANT 16: Xaa in position 16 represents a lysine amino acid bound on the nitrogen atom of its lateral chain to a -(TTDS)3-(gamma glutamic acid)4-Myristoyl (-(TTDS)3-(gE)4-Myr)
  VARIANT 21: Xaa in position 21 represents α-methyl-lysine (Mly)
  VARIANT 24: The peptide is substituted with an –NH2 group on its C-terminal extremity
LEGREKVRAXIXXEGXSTFSXRAK

SEQ ID NO: 98-99 - skipped (2 entries)

SEQ ID NO: 100 - protein, 24 aa, Artificial Sequence
  H2-relaxin A chain
  H2-relaxin A chain
  VARIANT 1: The peptide is substituted with a hydrogen atom (H) on its N-terminal extremity
QLYSALANKCCHVGCTKRSLARFC

SEQ ID NO: 101 - protein, 29 aa, Artificial Sequence
  H2-relaxin B chain
  H2-relaxin B chain
  VARIANT 1: The peptide is substituted with a hydrogen atom (H) on its N-terminal extremity
DSWMEEVIKLCGRELVRAQIAICGMSTWS

SEQ ID NO: 102 - protein, 27 aa, Artificial Sequence
  Peptide analogue of the B-chain of Relaxin-2 - comparison example
  Peptide analogue of the B-chain of Relaxin-2 - comparison example
  VARIANT 1: The peptide is substituted with a hydrogen atom (H) on its N-terminal extremity
  VARIANT 27: The peptide is substituted with an –NH2 group on its C-terminal extremity
VIKLSGRELVRAQIAISGMSTWSKRSL

SEQ ID NO: 103 - protein, 27 aa, Artificial Sequence
  Peptide analogue of the B-chain of Relaxin-2 - comparison example
  Peptide analogue of the B-chain of Relaxin-2 - comparison example
  VARIANT 1: The peptide is substituted with an acetyl (Ac) group on its N-terminal extremity
  VARIANT 27: The peptide is substituted with an –NH2 group on its C-terminal extremity
VIKLSGRELVRAQIAISGMSTWSKRSL

SEQ ID NO: 104 - protein, 27 aa, Artificial Sequence
  Peptide analogue of the B-chain of Relaxin-2 - comparison example
  Peptide analogue of the B-chain of Relaxin-2 - comparison example
  VARIANT 1: The peptide is substituted with an acetyl (Ac) group on its N-terminal extremity
  VARIANT 27: The peptide is substituted with an –NH2 group on its C-terminal extremity
VIKLSGRELVRAQIAISGMSTWSKKKK